European Patent Application EP 4 467 561 A1, published November 27, 2024. Title: TSP1 inhibitor. Applicant: DAIICHI SANKYO COMPANY, LIMITED. The sequence listing filed with the application follows.

SEQUENCE LISTING (166 sequences)

SEQ ID NO: 1 - protein, 12 aa, synthetic construct
  REGION 1..12: note = Peptide-1
  SITE 1: note = 3-(2-Naphthyl)-L-alanine
  SITE 3: note = L-Homocysteine
  SITE 5: note = (2S)-2-Amino-4-guanidino-butanoic acid
  SITE 8: note = L-Homocysteine
  SITE 11: note = L-Cyclopentylglycine
  SITE 12: note = Amidation of C-terminal carboxyl group
  SITE 1..12: note = Thiol group of cysteine is linked to N-terminal end of 3-(2-Naphthyl)-L-alanine via -CH2-CO-
  SITE 3..8: note = Thiol groups are linked as a disulfide
XRXGXNWXRWXC

SEQ ID NO: 2 - protein, 12 aa, synthetic construct
  REGION 1..12: note = Peptide-2
  SITE 1: note = 3-(2-Naphthyl)-L-alanine
  SITE 2: note = (2S)-2-Amino-4-guanidino-butanoic acid
  SITE 3: note = L-Homocysteine
  SITE 5: note = (2S)-2-Amino-4-guanidino-butanoic acid
  SITE 8: note = L-Homocysteine
  SITE 11: note = L-Cyclopentylglycine
  SITE 12: note = Amidation of C-terminal carboxyl group
  SITE 1..12: note = Thiol group of cysteine is linked to N-terminal end of 3-(2-Naphthyl)-L-alanine via -CH2-CO-
  SITE 3..8: note = Thiol groups are linked as a disulfide
XXXGXNWXRWXC

SEQ ID NO: 3 - protein, 12 aa, synthetic construct
  REGION 1..12: note = Peptide-3
  SITE 1: note = 3-(2-Naphthyl)-L-alanine
  SITE 2: note = L-Phenylglycine
  SITE 3: note = L-Homocysteine
  SITE 5: note = (2S)-2-Amino-4-guanidino-butanoic acid
  SITE 8: note = L-Homocysteine
  SITE 11: note = L-Cyclopentylglycine
  SITE 12: note = Amidation of C-terminal carboxyl group
  SITE 1..12: note = Thiol group of cysteine is linked to N-terminal end of 3-(2-Naphthyl)-L-alanine via -CH2-CO-
  SITE 3..8: note = Thiol groups are linked as a disulfide
XXXGXNWXRWXC

SEQ ID NO: 4 - protein, 12 aa, synthetic construct
  REGION 1..12: note = Peptide-4
  SITE 1: note = 3-(2-Naphthyl)-L-alanine
  SITE 3: note = L-Homocysteine
  SITE 5: note = (2S)-2-Amino-4-guanidino-butanoic acid
  SITE 8: note = L-Homocysteine
  SITE 9: note = L-Phenylglycine
  SITE 11: note = L-Cyclopentylglycine
  SITE 12: note = Amidation of C-terminal carboxyl group
  SITE 1..12: note = Thiol group of cysteine is linked to N-terminal end of 3-(2-Naphthyl)-L-alanine via -CH2-CO-
  SITE 3..8: note = Thiol groups are linked as a disulfide
XRXGXNWXXWXC

SEQ ID NO: 5 - protein, 12 aa, synthetic construct
  REGION 1..12: note = Peptide-5
  SITE 1: note = 3-(2-Naphthyl)-L-alanine
  SITE 3: note = L-Homocysteine
  SITE 5: note = (2S)-2-Amino-4-guanidino-butanoic acid
  SITE 8: note = L-Homocysteine
  SITE 9: note = L-4-Pyridylalanine
  SITE 11: note = L-Cyclopentylglycine
  SITE 12: note = Amidation of C-terminal carboxyl group
  SITE 1..12: note = Thiol group of cysteine is linked to N-terminal end of 3-(2-Naphthyl)-L-alanine via -CH2-CO-
  SITE 3..8: note = Thiol groups are linked as a disulfide
XRXGXNWXXWXC

SEQ ID NO: 6 - protein, 12 aa, synthetic construct
  REGION 1..12: note = Peptide-6
  SITE 1: note = 3-(2-Naphthyl)-L-alanine
  SITE 3: note = L-Homocysteine
  SITE 8: note = L-Homocysteine
  SITE 12: note = Amidation of C-terminal carboxyl group
  SITE 1..12: note = Thiol group of cysteine is linked to N-terminal end of 3-(2-Naphthyl)-L-alanine via -CH2-CO-
  SITE 3..8: note = Thiol groups are linked as a disulfide
XRXGRNWXVWVC

SEQ ID NO: 7 - protein, 12 aa, synthetic construct
  REGION 1..12: note = Peptide-7
  SITE 1: note = 3-(2-Naphthyl)-L-alanine
  SITE 3: note = L-Homocysteine
  SITE 8: note = L-Homocysteine
  SITE 11: note = L-Cyclopentylglycine
  SITE 12: note = Amidation of C-terminal carboxyl group
  SITE 1..12: note = Thiol group of cysteine is linked to N-terminal end of 3-(2-Naphthyl)-L-alanine via -CH2-CO-
  SITE 3..8: note = Thiol groups are linked as a disulfide
XRXGRNWXVWXC

SEQ ID NO: 8 - protein, 12 aa, synthetic construct
  REGION 1..12: note = Peptide-8
  SITE 1: note = 3-(2-Naphthyl)-L-alanine
  SITE 2: note = L-Tert-Leucine
  SITE 3: note = L-Homocysteine
  SITE 8: note = L-Homocysteine
  SITE 11: note = L-Cyclopentylglycine
  SITE 12: note = Amidation of C-terminal carboxyl group
  SITE 1..12: note = Thiol group of cysteine is linked to N-terminal end of 3-(2-Naphthyl)-L-alanine via -CH2-CO-
  SITE 3..8: note = Thiol groups are linked as a disulfide
XXXGRNWXRWXC

SEQ ID NO: 9 - protein, 12 aa, synthetic construct
  REGION 1..12: note = Peptide-9
  SITE 1: note = 3-(2-Naphthyl)-L-alanine
  SITE 3: note = L-Homocysteine
  SITE 5: note = (2S)-2-Amino-4-guanidino-butanoic acid
  SITE 8: note = L-Homocysteine
  SITE 11: note = L-Cyclopentylglycine
  SITE 12: note = Amidation of C-terminal carboxyl group
  SITE 1..12: note = Thiol group of cysteine is linked to N-terminal end of 3-(2-Naphthyl)-L-alanine via -CH2-CO-
  SITE 3..8: note = Thiol groups are linked as a disulfide
XRXGXDWXRWXC

SEQ ID NO: 10 - protein, 12 aa, synthetic construct
  REGION 1..12: note = Peptide-10
  SITE 1: note = 3-(2-Naphthyl)-L-alanine
  SITE 3: note = L-Homocysteine
  SITE 8: note = L-Homocysteine
  SITE 11: note = L-Cyclopentylglycine
  SITE 12: note = Amidation of C-terminal carboxyl group
  SITE 1..12: note = Thiol group of cysteine is linked to N-terminal end of 3-(2-Naphthyl)-L-alanine via -CH2-CO-
  SITE 3..8: note = Thiol groups are linked as a disulfide
XRXGRNWXRWXC

SEQ ID NO: 11 - protein, 12 aa, synthetic construct
  REGION 1..12: note = Peptide-11
  SITE 1: note = 3-(2-Naphthyl)-L-alanine
  SITE 3: note = L-Homocysteine
  SITE 8: note = L-Homocysteine
  SITE 11: note = L-Cyclopentylglycine
  SITE 12: note = Amidation of C-terminal carboxyl group
  SITE 1..12: note = Thiol group of cysteine is linked to N-terminal end of 3-(2-Naphthyl)-L-alanine via -CH2-CO-
  SITE 3..8: note = Thiol groups are linked as a disulfide
XRXGRDWXRWXC

SEQ ID NO: 12 - protein, 12 aa, synthetic construct
  REGION 1..12: note = Peptide-12
  SITE 1: note = 3-(2-Naphthyl)-L-alanine
  SITE 3: note = L-Homocysteine
  SITE 8: note = L-Homocysteine
  SITE 12: note = Amidation of C-terminal carboxyl group
  SITE 1..12: note = Thiol group of cysteine is linked to N-terminal end of 3-(2-Naphthyl)-L-alanine via -CH2-CO-
  SITE 3..8: note = Thiol groups are linked as a disulfide
XRXGRNWXRWVC

SEQ ID NO: 13 - protein, 21 aa, synthetic construct
  REGION 1..21: note = Peptide-13
  SITE 1: note = 3-(2-Naphthyl)-L-alanine
  SITE 3: note = L-Homocysteine
  SITE 5: note = (2S)-2-Amino-4-guanidino-butanoic acid
  SITE 8: note = L-Homocysteine
  SITE 11: note = L-Cyclopentylglycine
  SITE 20: note = 3-[2-[2-[2-[2-[2-[2-[2-[2-[2-[2-[2-(2-Aminoethoxy)ethoxy]ethoxy]ethoxy]ethoxy]ethoxy]ethoxy]ethoxy]ethoxy]ethoxy]ethoxy]ethoxy]propanoic acid
  SITE 1..12: note = Thiol group of cysteine is linked to N-terminal end of 3-(2-Naphthyl)-L-alanine via -CH2-CO-
  SITE 3..8: note = Thiol groups are linked as a disulfide
  SITE 21: note = Amidation of C-terminal carboxyl group
  SITE 21: note = Lysine side chain is modified with maleimide
XRXGXNWXRWXCGGGGDDDXK

SEQ ID NO: 14 - protein, 20 aa, synthetic construct
  REGION 1..20: note = Peptide-14
  SITE 1: note = 3-(2-Naphthyl)-L-alanine
  SITE 3: note = L-Homocysteine
  SITE 5: note = (2S)-2-Amino-4-guanidino-butanoic acid
  SITE 8: note = L-Homocysteine
  SITE 11: note = L-Cyclopentylglycine
  SITE 19: note = 3-[2-[2-[2-[2-[2-[2-[2-[2-[2-[2-[2-(2-Aminoethoxy)ethoxy]ethoxy]ethoxy]ethoxy]ethoxy]ethoxy]ethoxy]ethoxy]ethoxy]ethoxy]ethoxy]propanoic acid
  SITE 1..12: note = Thiol group of cysteine is linked to N-terminal end of 3-(2-Naphthyl)-L-alanine via -CH2-CO-
  SITE 3..8: note = Thiol groups are linked as a disulfide
  SITE 20: note = Amidation of C-terminal carboxyl group
  SITE 20: note = Lysine side chain is modified with maleimide
XRXGXDWXRWXCGGGGDDXK

SEQ ID NO: 15 - protein, 19 aa, synthetic construct
  REGION 1..19: note = Peptide-15
  SITE 1: note = 3-(2-Naphthyl)-L-alanine
  SITE 3: note = L-Homocysteine
  SITE 5: note = (2S)-2-Amino-4-guanidino-butanoic acid
  SITE 8: note = L-Homocysteine
  SITE 11: note = L-Cyclopentylglycine
  SITE 18: note = 3-[2-[2-[2-[2-[2-[2-[2-[2-[2-[2-[2-(2-Aminoethoxy)ethoxy]ethoxy]ethoxy]ethoxy]ethoxy]ethoxy]ethoxy]ethoxy]ethoxy]ethoxy]ethoxy]propanoic acid
  SITE 1..12: note = Thiol group of cysteine is linked to N-terminal end of 3-(2-Naphthyl)-L-alanine via -CH2-CO-
  SITE 3..8: note = Thiol groups are linked as a disulfide
  SITE 19: note = Lysine side chain is modified with maleimide
XRXGXDWXRWXCGGGGDXK

SEQ ID NO: 16 - protein, 22 aa, synthetic construct
  REGION 1..22: note = Peptide-16
  SITE 1: note = 3-(2-Naphthyl)-L-alanine
  SITE 3: note = L-Homocysteine
  SITE 8: note = L-Homocysteine
  SITE 11: note = L-Cyclopentylglycine
  SITE 19: note = (2S)-6-amino-2-[[2-[2-[2-[2-[2-[2-[2-[2-[2-[2-(2-methoxyethoxy)ethoxy]ethoxy]ethoxy]ethoxy]ethoxy]ethoxy]ethoxy]ethoxy]ethoxy]acetyl]amino]hexanoic acid
  REGION 20..21: note = 3-[2-[2-[2-[2-[2-[2-[2-[2-[2-[2-[2-(2-Aminoethoxy)ethoxy]ethoxy]ethoxy]ethoxy]ethoxy]ethoxy]ethoxy]ethoxy]ethoxy]ethoxy]ethoxy]propanoic acid
  SITE 1..12: note = Thiol group of cysteine is linked to N-terminal end of 3-(2-Naphthyl)-L-alanine via -CH2-CO-
  SITE 3..8: note = Thiol groups are linked as a disulfide
  SITE 22: note = Amidation of C-terminal carboxyl group
  SITE 22: note = Lysine side chain is modified with maleimide
XRXGRDWXRWXCGGGGDDXXXK

SEQ ID NO: 17 - protein, 22 aa, synthetic construct
  REGION 1..22: note = Peptide-17
  SITE 1: note = 3-(2-Naphthyl)-L-alanine
  SITE 3: note = L-Homocysteine
  SITE 8: note = L-Homocysteine
  SITE 11: note = L-Cyclopentylglycine
  REGION 19..20: note = 3-[2-[2-[2-[2-[2-[2-[2-[2-[2-[2-[2-(2-Aminoethoxy)ethoxy]ethoxy]ethoxy]ethoxy]ethoxy]ethoxy]ethoxy]ethoxy]ethoxy]ethoxy]ethoxy]propanoic acid
  SITE 21: note = (2S)-6-amino-2-[[2-[2-[2-[2-[2-[2-[2-[2-[2-[2-(2-methoxyethoxy)ethoxy]ethoxy]ethoxy]ethoxy]ethoxy]ethoxy]ethoxy]ethoxy]ethoxy]acetyl]amino]hexanoic acid
  SITE 1..12: note = Thiol group of cysteine is linked to N-terminal end of 3-(2-Naphthyl)-L-alanine via -CH2-CO-
  SITE 3..8: note = Thiol groups are linked as a disulfide
  SITE 22: note = Amidation of C-terminal carboxyl group
  SITE 22: note = Lysine side chain is modified with maleimide
XRXGRDWXRWXCGSGSDDXXXK

SEQ ID NO: 18 - protein, 22 aa, synthetic construct
  REGION 1..22: note = Peptide-18
  SITE 1: note = 3-(2-Naphthyl)-L-alanine
  SITE 3: note = L-Homocysteine
  SITE 8: note = L-Homocysteine
  SITE 11: note = L-Cyclopentylglycine
  REGION 19..20: note = 3-[2-[2-[2-[2-[2-[2-[2-[2-[2-[2-[2-(2-Aminoethoxy)ethoxy]ethoxy]ethoxy]ethoxy]ethoxy]ethoxy]ethoxy]ethoxy]ethoxy]ethoxy]ethoxy]propanoic acid
  SITE 21: note = (2S)-6-amino-2-[[2-[2-[2-[2-[2-[2-[2-[2-[2-[2-(2-methoxyethoxy)ethoxy]ethoxy]ethoxy]ethoxy]ethoxy]ethoxy]ethoxy]ethoxy]ethoxy]acetyl]amino]hexanoic acid
  SITE 1..12: note = Thiol group of cysteine is linked to N-terminal end of 3-(2-Naphthyl)-L-alanine via -CH2-CO-
  SITE 3..8: note = Thiol groups are linked as a disulfide
  SITE 22: note = Amidation of C-terminal carboxyl group
  SITE 22: note = Lysine side chain is modified with maleimide
XRXGRDWXRWXCGGGGDDXXXK

SEQ ID NO: 19 - protein, 22 aa, synthetic construct
  REGION 1..22: note = Peptide-19
  SITE 1: note = 3-(2-Naphthyl)-L-alanine
  SITE 3: note = L-Homocysteine
  SITE 8: note = L-Homocysteine
  SITE 11: note = L-Cyclopentylglycine
  SITE 19: note = 3-[2-[2-[2-[2-[2-[2-[2-[2-[2-[2-[2-(2-Aminoethoxy)ethoxy]ethoxy]ethoxy]ethoxy]ethoxy]ethoxy]ethoxy]ethoxy]ethoxy]ethoxy]ethoxy]propanoic acid
  SITE 20: note = (2S)-6-amino-2-[[2-[2-[2-[2-[2-[2-[2-[2-[2-[2-(2-methoxyethoxy)ethoxy]ethoxy]ethoxy]ethoxy]ethoxy]ethoxy]ethoxy]ethoxy]ethoxy]acetyl]amino]hexanoic acid
  SITE 21: note = 3-[2-[2-[2-[2-[2-[2-[2-[2-[2-[2-[2-(2-Aminoethoxy)ethoxy]ethoxy]ethoxy]ethoxy]ethoxy]ethoxy]ethoxy]ethoxy]ethoxy]ethoxy]ethoxy]propanoic acid
  SITE 1..12: note = Thiol group of cysteine is linked to N-terminal end of 3-(2-Naphthyl)-L-alanine via -CH2-CO-
  SITE 3..8: note = Thiol groups are linked as a disulfide
  SITE 22: note = Amidation of C-terminal carboxyl group
  SITE 22: note = Lysine side chain is modified with maleimide
XRXGRDWXRWXCGGGGDDXXXK

SEQ ID NO: 20 - protein, 22 aa, synthetic construct
  REGION 1..22: note = Peptide-20
  SITE 1: note = 3-(2-Naphthyl)-L-alanine
  SITE 3: note = L-Homocysteine
  SITE 8: note = L-Homocysteine
  SITE 11: note = L-Cyclopentylglycine
  REGION 13..16: note = MeGly
  SITE 19: note = (2S)-6-amino-2-[[2-[2-[2-[2-[2-[2-[2-[2-[2-[2-(2-methoxyethoxy)ethoxy]ethoxy]ethoxy]ethoxy]ethoxy]ethoxy]ethoxy]ethoxy]ethoxy]acetyl]amino]hexanoic acid
  REGION 20..21: note = 3-[2-[2-[2-[2-[2-[2-[2-[2-[2-[2-[2-(2-Aminoethoxy)ethoxy]ethoxy]ethoxy]ethoxy]ethoxy]ethoxy]ethoxy]ethoxy]ethoxy]ethoxy]ethoxy]propanoic acid
  SITE 1..12: note = Thiol group of cysteine is linked to N-terminal end of 3-(2-Naphthyl)-L-alanine via -CH2-CO-
  SITE 3..8: note = Thiol groups are linked as a disulfide
  SITE 22: note = Amidation of C-terminal carboxyl group
  SITE 22: note = Lysine side chain is modified with maleimide
XRXGRDWXRWXCXXXXDDXXXK

SEQ ID NO: 21 - protein, 22 aa, synthetic construct
  REGION 1..22: note = Peptide-21
  SITE 1: note = 3-(2-Naphthyl)-L-alanine
  SITE 3: note = L-Homocysteine
  SITE 8: note = L-Homocysteine
  SITE 11: note = L-Cyclopentylglycine
  REGION 13..16: note = MeGly
  SITE 19: note = 3-[2-[2-[2-[2-[2-[2-[2-[2-[2-[2-[2-(2-Aminoethoxy)ethoxy]ethoxy]ethoxy]ethoxy]ethoxy]ethoxy]ethoxy]ethoxy]ethoxy]ethoxy]ethoxy]propanoic acid
  SITE 20: note = (2S)-6-amino-2-[[2-[2-[2-[2-[2-[2-[2-[2-[2-[2-(2-methoxyethoxy)ethoxy]ethoxy]ethoxy]ethoxy]ethoxy]ethoxy]ethoxy]ethoxy]ethoxy]acetyl]amino]hexanoic acid
  SITE 21: note = 3-[2-[2-[2-[2-[2-[2-[2-[2-[2-[2-[2-(2-Aminoethoxy)ethoxy]ethoxy]ethoxy]ethoxy]ethoxy]ethoxy]ethoxy]ethoxy]ethoxy]ethoxy]ethoxy]propanoic acid
  SITE 1..12: note = Thiol group of cysteine is linked to N-terminal end of 3-(2-Naphthyl)-L-alanine via -CH2-CO-
  SITE 3..8: note = Thiol groups are linked as a disulfide
  SITE 22: note = Amidation of C-terminal carboxyl group
  SITE 22: note = Lysine side chain is modified with maleimide
XRXGRDWXRWXCXXXXDDXXXK

SEQ ID NO: 22 - protein, 22 aa, synthetic construct
  REGION 1..22: note = Peptide-22
  SITE 1: note = 3-(2-Naphthyl)-L-alanine
  SITE 3: note = L-Homocysteine
  SITE 8: note = L-Homocysteine
  SITE 11: note = L-Cyclopentylglycine
  SITE 19: note = (2S)-6-amino-2-[[2-[2-[2-[2-[2-[2-[2-[2-[2-[2-(2-methoxyethoxy)ethoxy]ethoxy]ethoxy]ethoxy]ethoxy]ethoxy]ethoxy]ethoxy]ethoxy]acetyl]amino]hexanoic acid
  REGION 20..21: note = 3-[2-[2-[2-[2-[2-[2-[2-[2-[2-[2-[2-(2-Aminoethoxy)ethoxy]ethoxy]ethoxy]ethoxy]ethoxy]ethoxy]ethoxy]ethoxy]ethoxy]ethoxy]ethoxy]propanoic acid
  SITE 1..12: note = Thiol group of cysteine is linked to N-terminal end of 3-(2-Naphthyl)-L-alanine via -CH2-CO-
  SITE 3..8: note = Thiol groups are linked as a disulfide
  SITE 22: note = Amidation of C-terminal carboxyl group
  SITE 22: note = Lysine side chain is modified with maleimide
XRXGRDWXRWXCGSGSDDXXXK

SEQ ID NO: 23 - protein, 22 aa, synthetic construct
  REGION 1..22: note = Peptide-23
  SITE 1: note = 3-(2-Naphthyl)-L-alanine
  SITE 3: note = L-Homocysteine
  SITE 8: note = L-Homocysteine
  SITE 11: note = L-Cyclopentylglycine
  SITE 19: note = 3-[2-[2-[2-[2-[2-[2-[2-[2-[2-[2-[2-(2-Aminoethoxy)ethoxy]ethoxy]ethoxy]ethoxy]ethoxy]ethoxy]ethoxy]ethoxy]ethoxy]ethoxy]ethoxy]propanoic acid
  SITE 20: note = (2S)-6-amino-2-[[2-[2-[2-[2-[2-[2-[2-[2-[2-[2-(2-methoxyethoxy)ethoxy]ethoxy]ethoxy]ethoxy]ethoxy]ethoxy]ethoxy]ethoxy]ethoxy]acetyl]amino]hexanoic acid
  SITE 21: note = 3-[2-[2-[2-[2-[2-[2-[2-[2-[2-[2-[2-(2-Aminoethoxy)ethoxy]ethoxy]ethoxy]ethoxy]ethoxy]ethoxy]ethoxy]ethoxy]ethoxy]ethoxy]ethoxy]propanoic acid
  SITE 1..12: note = Thiol group of cysteine is linked to N-terminal end of 3-(2-Naphthyl)-L-alanine via -CH2-CO-
  SITE 3..8: note = Thiol groups are linked as a disulfide
  SITE 22: note = Amidation of C-terminal carboxyl group
  SITE 22: note = Lysine side chain is modified with maleimide
XRXGRDWXRWXCGSGSDDXXXK

SEQ ID NO: 24 - protein, 22 aa, synthetic construct
  REGION 1..22: note = Peptide-24
  SITE 1: note = 3-(2-Naphthyl)-L-alanine
  SITE 3: note = L-Homocysteine
  SITE 8: note = L-Homocysteine
  SITE 11: note = L-Cyclopentylglycine
  REGION 13..16: note = MeGly
  REGION 19..20: note = 3-[2-[2-[2-[2-[2-[2-[2-[2-[2-[2-[2-(2-Aminoethoxy)ethoxy]ethoxy]ethoxy]ethoxy]ethoxy]ethoxy]ethoxy]ethoxy]ethoxy]ethoxy]ethoxy]propanoic acid
  SITE 21: note = (2S)-6-amino-2-[[2-[2-[2-[2-[2-[2-[2-[2-[2-[2-(2-methoxyethoxy)ethoxy]ethoxy]ethoxy]ethoxy]ethoxy]ethoxy]ethoxy]ethoxy]ethoxy]acetyl]amino]hexanoic acid
  SITE 1..12: note = Thiol group of cysteine is linked to N-terminal end of 3-(2-Naphthyl)-L-alanine via -CH2-CO-
  SITE 3..8: note = Thiol groups are linked as a disulfide
  SITE 22: note = Amidation of C-terminal carboxyl group
  SITE 22: note = Lysine side chain is modified with maleimide
XRXGRDWXRWXCXXXXDDXXXK

SEQ ID NO: 25 - protein, 18 aa, synthetic construct
  REGION 1..18: note = Peptide-25
  SITE 1: note = 3-(2-Naphthyl)-L-alanine
  SITE 17: note = 3-[2-[2-[2-[2-[2-[2-[2-[2-[2-[2-[2-(2-Aminoethoxy)ethoxy]ethoxy]ethoxy]ethoxy]ethoxy]ethoxy]ethoxy]ethoxy]ethoxy]ethoxy]ethoxy]propanoic acid
  SITE 1..12: note = Thiol group of cysteine is linked to N-terminal end of 3-(2-Naphthyl)-L-alanine via -CH2-CO-
  SITE 18: note = Amidation of C-terminal carboxyl group
  SITE 18: note = Lysine side chain is modified with maleimide
XRSGRNWVVWVCGGGGXK

SEQ ID NO: 26 - protein, 18 aa, synthetic construct
  REGION 1..18: note = Peptide-26
  SITE 1: note = 3-(2-Naphthyl)-L-alanine
  SITE 17: note = 3-[2-[2-[2-[2-[2-[2-[2-[2-[2-[2-[2-(2-Aminoethoxy)ethoxy]ethoxy]ethoxy]ethoxy]ethoxy]ethoxy]ethoxy]ethoxy]ethoxy]ethoxy]ethoxy]propanoic acid
  SITE 1..12: note = Thiol group of cysteine is linked to N-terminal end of 3-(2-Naphthyl)-L-alanine via -CH2-CO-
  SITE 18: note = Amidation of C-terminal carboxyl group
  SITE 18: note = Lysine side chain is modified with maleimide
XRSGRNWVRWVCGGGGXK

SEQ ID NO: 27 - protein, 20 aa, synthetic construct
  REGION 1..20: note = Peptide-27
  SITE 1: note = 3-(2-Naphthyl)-L-alanine
  SITE 5: note = (2S)-2-Amino-4-guanidino-butanoic acid
  SITE 11: note = L-Cyclopentylglycine
  SITE 19: note = 3-[2-[2-[2-[2-[2-[2-[2-[2-[2-[2-[2-(2-Aminoethoxy)ethoxy]ethoxy]ethoxy]ethoxy]ethoxy]ethoxy]ethoxy]ethoxy]ethoxy]ethoxy]ethoxy]propanoic acid
  SITE 1..12: note = Thiol group of cysteine is linked to N-terminal end of 3-(2-Naphthyl)-L-alanine via -CH2-CO-
  SITE 20: note = Amidation of C-terminal carboxyl group
  SITE 20: note = Lysine side chain is modified with maleimide
XRSGXNWVRWXCGGGGDDXK

SEQ ID NO: 28 - protein, 18 aa, synthetic construct
  REGION 1..18: note = Peptide-28
  SITE 1: note = 3-(2-Naphthyl)-L-alanine
  SITE 5: note = (2S)-2-Amino-4-guanidino-butanoic acid
  SITE 11: note = L-Cyclopentylglycine
  SITE 17: note = 3-[2-[2-[2-[2-[2-[2-[2-[2-[2-[2-[2-(2-Aminoethoxy)ethoxy]ethoxy]ethoxy]ethoxy]ethoxy]ethoxy]ethoxy]ethoxy]ethoxy]ethoxy]ethoxy]propanoic acid
  SITE 1..12: note = Thiol group of cysteine is linked to N-terminal end of 3-(2-Naphthyl)-L-alanine via -CH2-CO-
  SITE 18: note = Amidation of C-terminal carboxyl group
  SITE 18: note = Lysine side chain is modified with maleimide
XRSGXNWVRWXCGGGGXK

SEQ ID NO: 29 - protein, 20 aa, synthetic construct
  REGION 1..20: note = Peptide-29
  SITE 1: note = 3-(2-Naphthyl)-L-alanine
  SITE 5: note = (2S)-2-Amino-4-guanidino-butanoic acid
  SITE 11: note = L-Cyclopentylglycine
  SITE 17: note = 3-[2-[2-[2-[2-[2-[2-[2-[2-[2-[2-[2-(2-Aminoethoxy)ethoxy]ethoxy]ethoxy]ethoxy]ethoxy]ethoxy]ethoxy]ethoxy]ethoxy]ethoxy]ethoxy]propanoic acid
  SITE 1..12: note = Thiol group of cysteine is linked to N-terminal end of 3-(2-Naphthyl)-L-alanine via -CH2-CO-
  SITE 20: note = Amidation of C-terminal carboxyl group
  SITE 20: note = Lysine side chain is modified with maleimide
XRSGXNWVRWXCGGGGXDDK

SEQ ID NO: 30 - protein, 20 aa, synthetic construct
  REGION 1..20: note = Peptide-30
  SITE 1: note = 3-(2-Naphthyl)-L-alanine
  SITE 5: note = (2S)-2-Amino-4-guanidino-butanoic acid
  SITE 11: note = L-Cyclopentylglycine
  REGION 13..16: note = bAla
  SITE 19: note = 3-[2-[2-[2-[2-[2-[2-[2-[2-[2-[2-[2-(2-Aminoethoxy)ethoxy]ethoxy]ethoxy]ethoxy]ethoxy]ethoxy]ethoxy]ethoxy]ethoxy]ethoxy]ethoxy]propanoic acid
  SITE 1..12: note = Thiol group of cysteine is linked to N-terminal end of 3-(2-Naphthyl)-L-alanine via -CH2-CO-
  SITE 20: note = Amidation of C-terminal carboxyl group
  SITE 20: note = Lysine side chain is modified with maleimide
XRSGXNWVRWXCXXXXDDXK

SEQ ID NO: 31 - protein, 20 aa, synthetic construct
  REGION 1..20: note = Peptide-31
  SITE 1: note = 3-(2-Naphthyl)-L-alanine
  SITE 5: note = (2S)-2-Amino-4-guanidino-butanoic acid
  SITE 11: note = L-Cyclopentylglycine
  REGION 17..18: note = D-Aspartic acid
  SITE 19: note = 3-[2-[2-[2-[2-[2-[2-[2-[2-[2-[2-[2-(2-Aminoethoxy)ethoxy]ethoxy]ethoxy]ethoxy]ethoxy]ethoxy]ethoxy]ethoxy]ethoxy]ethoxy]ethoxy]propanoic acid
  SITE 1..12: note = Thiol group of cysteine is linked to N-terminal end of 3-(2-Naphthyl)-L-alanine via -CH2-CO-
  SITE 20: note = Amidation of C-terminal carboxyl group
  SITE 20: note = Lysine side chain is modified with maleimide
XRSGXNWVRWXCGGGGXXXK

SEQ ID NO: 32 - protein, 20 aa, synthetic construct
  REGION 1..20: note = Peptide-32
  SITE 1: note = 3-(2-Naphthyl)-L-alanine
  SITE 5: note = (2S)-2-Amino-4-guanidino-butanoic acid
  SITE 11: note = L-Cyclopentylglycine
  REGION 13..16: note = bAla
  REGION 17..18: note = D-Aspartic acid
  SITE 19: note = 3-[2-[2-[2-[2-[2-[2-[2-[2-[2-[2-[2-(2-Aminoethoxy)ethoxy]ethoxy]ethoxy]ethoxy]ethoxy]ethoxy]ethoxy]ethoxy]ethoxy]ethoxy]ethoxy]propanoic acid
  SITE 1..12: note = Thiol group of cysteine is linked to N-terminal end of 3-(2-Naphthyl)-L-alanine via -CH2-CO-
  SITE 20: note = Amidation of C-terminal carboxyl group
  SITE 20: note = Lysine side chain is modified with maleimide
XRSGXNWVRWXCXXXXXXXK

SEQ ID NO: 33 - protein, 18 aa, synthetic construct
  REGION 1..18: note = Peptide-33
  SITE 1: note = 3-(2-Naphthyl)-L-alanine
  SITE 8: note = Nle
  SITE 11: note = L-Alpha-cyclohexylglycine
  SITE 17: note = 3-[2-[2-[2-[2-[2-[2-[2-[2-[2-[2-[2-(2-Aminoethoxy)ethoxy]ethoxy]ethoxy]ethoxy]ethoxy]ethoxy]ethoxy]ethoxy]ethoxy]ethoxy]ethoxy]propanoic acid
  SITE 1..12: note = Thiol group of cysteine is linked to N-terminal end of 3-(2-Naphthyl)-L-alanine via -CH2-CO-
  SITE 18: note = Amidation of C-terminal carboxyl group
  SITE 18: note = Lysine side chain is modified with maleimide
XRSGRNWXVWXCGGGGXK

SEQ ID NO: 34 - protein, 20 aa, synthetic construct
  REGION 1..20: note = Peptide-34
  SITE 1: note = 3-(2-Naphthyl)-L-alanine
  SITE 8: note = Nle
  SITE 11: note = L-Alpha-cyclohexylglycine
  SITE 19: note = 3-[2-[2-[2-[2-[2-[2-[2-[2-[2-[2-[2-(2-Aminoethoxy)ethoxy]ethoxy]ethoxy]ethoxy]ethoxy]ethoxy]ethoxy]ethoxy]ethoxy]ethoxy]ethoxy]propanoic acid
  SITE 1..12: note = Thiol group of cysteine is linked to N-terminal end of 3-(2-Naphthyl)-L-alanine via -CH2-CO-
  SITE 20: note = Amidation of C-terminal carboxyl group
  SITE 20: note = Lysine side chain is modified with maleimide
XRSGRNWXVWXCGGGGDDXK

SEQ ID NO: 35 - protein, 19 aa, synthetic construct
  REGION 1..19: note = Peptide-35
  SITE 1: note = 3-(2-Naphthyl)-L-alanine
  SITE 5: note = (2S)-2-Amino-4-guanidino-butanoic acid
  SITE 11: note = L-Cyclopentylglycine
  SITE 18: note = 3-[2-[2-[2-[2-[2-[2-[2-[2-[2-[2-[2-(2-Aminoethoxy)ethoxy]ethoxy]ethoxy]ethoxy]ethoxy]ethoxy]ethoxy]ethoxy]ethoxy]ethoxy]ethoxy]propanoic acid
  SITE 1..12: note = Thiol group of cysteine is linked to N-terminal end of 3-(2-Naphthyl)-L-alanine via -CH2-CO-
  SITE 19: note = Amidation of C-terminal carboxyl group
  SITE 19: note = Lysine side chain is modified with maleimide
XRSGXDWVRWXCGGGGDXK

SEQ ID NO: 36 - protein, 18 aa, synthetic construct
  REGION 1..18: note = Peptide-36
  SITE 1: note = 3-(2-Naphthyl)-L-alanine
  SITE 5: note = (2S)-2-Amino-4-guanidino-butanoic acid
  SITE 11: note = L-Cyclopentylglycine
  SITE 17: note = 3-[2-[2-[2-[2-[2-[2-[2-[2-[2-[2-[2-(2-Aminoethoxy)ethoxy]ethoxy]ethoxy]ethoxy]ethoxy]ethoxy]ethoxy]ethoxy]ethoxy]ethoxy]ethoxy]propanoic acid
  SITE 1..12: note = Thiol group of cysteine is linked to N-terminal end of 3-(2-Naphthyl)-L-alanine via -CH2-CO-
  SITE 18: note = Lysine side chain is modified with maleimide
XRSGXDWVRWXCGGGGXK

SEQ ID NO: 37 - protein, 18 aa, synthetic construct
  REGION 1..18: note = Peptide-37
  SITE 1: note = 3-(2-Naphthyl)-L-alanine
  SITE 5: note = (2S)-2-Amino-4-guanidino-butanoic acid
  SITE 8: note = Nle
  SITE 11: note = L-Alpha-cyclohexylglycine
  SITE 17: note = 3-[2-[2-[2-[2-[2-[2-[2-[2-[2-[2-[2-(2-Aminoethoxy)ethoxy]ethoxy]ethoxy]ethoxy]ethoxy]ethoxy]ethoxy]ethoxy]ethoxy]ethoxy]ethoxy]propanoic acid
  SITE 1..12: note = Thiol group of cysteine is linked to N-terminal end of 3-(2-Naphthyl)-L-alanine via -CH2-CO-
  SITE 18: note = Amidation of C-terminal carboxyl group
  SITE 18: note = Lysine side chain is modified with maleimide
XRSGXNWXVWXCGGGGXK

SEQ ID NO: 38 - protein, 20 aa, synthetic construct
  REGION 1..20: note = Peptide-38
  SITE 1: note = 3-(2-Naphthyl)-L-alanine
  SITE 5: note = (2S)-2-Amino-4-guanidino-butanoic acid
  SITE 8: note = Nle
  SITE 11: note = L-Alpha-cyclohexylglycine
  SITE 19: note = 3-[2-[2-[2-[2-[2-[2-[2-[2-[2-[2-[2-(2-Aminoethoxy)ethoxy]ethoxy]ethoxy]ethoxy]ethoxy]ethoxy]ethoxy]ethoxy]ethoxy]ethoxy]ethoxy]propanoic acid
  SITE 1..12: note = Thiol group of cysteine is linked to N-terminal end of 3-(2-Naphthyl)-L-alanine via -CH2-CO-
  SITE 20: note = Amidation of C-terminal carboxyl group
  SITE 20: note = Lysine side chain is modified with maleimide
XRSGXNWXVWXCGGGGDDXK

SEQ ID NO: 39 - protein, 20 aa, synthetic construct
  REGION 1..20: note = Peptide-39
  SITE 1: note = 3-(2-Naphthyl)-L-alanine
  SITE 5: note = (2S)-2-Amino-4-guanidino-butanoic acid
  SITE 8: note = Nle
  SITE 11: note = L-Alpha-cyclohexylglycine
  SITE 19: note = 3-[2-[2-[2-[2-[2-[2-[2-[2-[2-[2-[2-(2-Aminoethoxy)ethoxy]ethoxy]ethoxy]ethoxy]ethoxy]ethoxy]ethoxy]ethoxy]ethoxy]ethoxy]ethoxy]propanoic acid
  SITE 1..12: note = Thiol group of cysteine is linked to N-terminal end of 3-(2-Naphthyl)-L-alanine via -CH2-CO-
  SITE 20: note = Amidation of C-terminal carboxyl group
  SITE 20: note = Lysine side chain is modified with maleimide
XRSGXNWXRWXCGGGGDDXK

SEQ ID NO: 40 - protein, 19 aa, synthetic construct
  REGION 1..19: note = Peptide-40
  SITE 1: note = 3-(2-Naphthyl)-L-alanine
  SITE 5: note = (2S)-2-Amino-4-guanidino-butanoic acid
  SITE 8: note = Nle
  SITE 11: note = L-Cyclopentylglycine
  SITE 18: note = 3-[2-[2-[2-[2-[2-[2-[2-[2-[2-[2-[2-(2-Aminoethoxy)ethoxy]ethoxy]ethoxy]ethoxy]ethoxy]ethoxy]ethoxy]ethoxy]ethoxy]ethoxy]ethoxy]propanoic acid
  SITE 1..12: note = Thiol group of cysteine is linked to N-terminal end of 3-(2-Naphthyl)-L-alanine via -CH2-CO-
  SITE 19: note = Amidation of C-terminal carboxyl group
  SITE 19: note = Lysine side chain is modified with maleimide
XRSGXDWXRWXCGGGGDXK

SEQ ID NO: 41 - protein, 20 aa, synthetic construct
  REGION 1..20: note = Peptide-41
  SITE 1: note = 3-(2-Naphthyl)-L-alanine
  SITE 5: note = (2S)-2-Amino-4-guanidino-butanoic acid
  SITE 8: note = Nle
  SITE 11: note = L-Cyclopentylglycine
  SITE 17: note = 3-[2-[2-[2-[2-[2-[2-[2-[2-[2-[2-[2-(2-Aminoethoxy)ethoxy]ethoxy]ethoxy]ethoxy]ethoxy]ethoxy]ethoxy]ethoxy]ethoxy]ethoxy]ethoxy]propanoic acid
  SITE 1..12: note = Thiol group of cysteine is linked to N-terminal end of 3-(2-Naphthyl)-L-alanine via -CH2-CO-
  SITE 20: note = Amidation of C-terminal carboxyl group
  SITE 20: note = Lysine side chain is modified with maleimide
XRSGXNWXRWXCGGGGXDDK

SEQ ID NO: 42 - protein, 19 aa, synthetic construct
  REGION 1..19: note = Peptide-42
  SITE 1: note = 3-(2-Naphthyl)-L-alanine
  SITE 5: note = (2S)-2-Amino-4-guanidino-butanoic acid
  SITE 8: note = Nle
  SITE 11: note = L-Cyclopentylglycine
  SITE 17: note = 3-[2-[2-[2-[2-[2-[2-[2-[2-[2-[2-[2-(2-Aminoethoxy)ethoxy]ethoxy]ethoxy]ethoxy]ethoxy]ethoxy]ethoxy]ethoxy]ethoxy]ethoxy]ethoxy]propanoic acid
  SITE 1..12: note = Thiol group of cysteine is linked to N-terminal end of 3-(2-Naphthyl)-L-alanine via -CH2-CO-
  SITE 19: note = Amidation of C-terminal carboxyl group
  SITE 19: note = Lysine side chain is modified with maleimide
XRSGXDWXRWXCGGGGXDK

SEQ ID NO: 43 - protein, 20 aa, synthetic construct
  REGION 1..20: note = Peptide-43
  SITE 1: note = 3-(2-Naphthyl)-L-alanine
  SITE 5: note = (2S)-2-Amino-4-guanidino-butanoic acid
  SITE 8: note = Nle
  SITE 11: note = L-Alpha-cyclohexylglycine
  SITE 19: note = 3-[2-[2-[2-[2-[2-[2-[2-[2-[2-[2-[2-[2-[2-[2-[2-[2-[2-[2-[2-[2-[2-[2-[2-(2-Aminoethoxy)ethoxy]ethoxy]ethoxy]ethoxy]ethoxy]ethoxy]ethoxy]ethoxy]ethoxy]ethoxy]ethoxy]ethoxy]ethoxy]ethoxy]ethoxy]ethoxy]ethoxy]ethoxy]ethoxy]ethoxy]ethoxy]ethoxy]ethoxy]propanoic acid
  SITE 1..12: note = Thiol group of cysteine is linked to N-terminal end of 3-(2-Naphthyl)-L-alanine via -CH2-CO-
  SITE 20: note = Amidation of C-terminal carboxyl group
  SITE 20: note = Lysine side chain is modified with maleimide
XRSGXNWXRWXCGGGGDDXK

SEQ ID NO: 44 - protein, 21 aa, synthetic construct
  REGION 1..21: note = Peptide-44
  SITE 1: note = 3-(2-Naphthyl)-L-alanine
  SITE 5: note = (2S)-2-Amino-4-guanidino-butanoic acid
  SITE 8: note = Nle
  SITE 11: note = L-Alpha-cyclohexylglycine
  REGION 19..20: note = 3-[2-[2-[2-[2-[2-[2-[2-[2-[2-[2-[2-(2-Aminoethoxy)ethoxy]ethoxy]ethoxy]ethoxy]ethoxy]ethoxy]ethoxy]ethoxy]ethoxy]ethoxy]ethoxy]propanoic acid
  SITE 1..12: note = Thiol group of cysteine is linked to N-terminal end of 3-(2-Naphthyl)-L-alanine via -CH2-CO-
  SITE 21: note = Amidation of C-terminal carboxyl group
  SITE 21: note = Lysine side chain is modified with maleimide
XRSGXNWXRWXCGGGGDDXXK

SEQ ID NO: 45 - protein, 21 aa, synthetic construct
  REGION 1..21: note = Peptide-45
  SITE 1: note = 3-(2-Naphthyl)-L-alanine
  SITE 5: note = (2S)-2-Amino-4-guanidino-butanoic acid
  SITE 8: note = Nle
  SITE 11: note = L-Alpha-cyclohexylglycine
  REGION 13..16: note = MeGly
  REGION 19..20: note = 3-[2-[2-[2-[2-[2-[2-[2-[2-[2-[2-[2-(2-Aminoethoxy)ethoxy]ethoxy]ethoxy]ethoxy]ethoxy]ethoxy]ethoxy]ethoxy]ethoxy]ethoxy]ethoxy]propanoic acid
  SITE 1..12: note = Thiol group of cysteine is linked to N-terminal end of 3-(2-Naphthyl)-L-alanine via -CH2-CO-
  SITE 21: note = Amidation of C-terminal carboxyl group
  SITE 21: note = Lysine side chain is modified with maleimide
XRSGXNWXRWXCXXXXDDXXK

SEQ ID NO: 46 - protein, 21 aa, synthetic construct
  REGION 1..21: note = Peptide-46
  SITE 1: note = 3-(2-Naphthyl)-L-alanine
  SITE 5: note = (2S)-2-Amino-4-guanidino-butanoic acid
  SITE 8: note = Nle
  SITE 11: note = L-Alpha-cyclohexylglycine
  REGION 19..20: note = 3-[2-[2-[2-[2-[2-[2-[2-[2-[2-[2-[2-(2-Aminoethoxy)ethoxy]ethoxy]ethoxy]ethoxy]ethoxy]ethoxy]ethoxy]ethoxy]ethoxy]ethoxy]ethoxy]propanoic acid
  SITE 1..12: note = Thiol group of cysteine is linked to N-terminal end of 3-(2-Naphthyl)-L-alanine via -CH2-CO-
  SITE 21: note = Amidation of C-terminal carboxyl group
  SITE 21: note = Lysine side chain is modified with maleimide
XRSGXNWXRWXCGSGSDDXXK

SEQ ID NO: 47 - protein, 21 aa, synthetic construct
  REGION 1..21: note = Peptide-47
  SITE 1: note = 3-(2-Naphthyl)-L-alanine
  SITE 5: note = (2S)-2-Amino-4-guanidino-butanoic acid
  SITE 8: note = Nle
  SITE 11: note = L-Alpha-cyclohexylglycine
  REGION 19..20: note = 3-[2-[2-[2-[2-[2-[2-[2-[2-[2-[2-[2-(2-Aminoethoxy)ethoxy]ethoxy]ethoxy]ethoxy]ethoxy]ethoxy]ethoxy]ethoxy]ethoxy]ethoxy]ethoxy]propanoic acid
  SITE 1..12: note = Thiol group of cysteine is linked to N-terminal end of 3-(2-Naphthyl)-L-alanine via -CH2-CO-
  SITE 21: note = Amidation of C-terminal carboxyl group
  SITE 21: note = Lysine side chain is modified with maleimide
XRSGXNWXRWXCGGEGGEXXK

SEQ ID NO: 48 - protein, 21 aa, synthetic construct
  REGION 1..21: note = Peptide-48
  SITE 1: note = 3-(2-Naphthyl)-L-alanine
  SITE 5: note = (2S)-2-Amino-4-guanidino-butanoic acid
  SITE 8: note = Nle
  SITE 11: note = L-Alpha-cyclohexylglycine
  SITE 18: note = 3-[2-[2-[2-[2-[2-[2-[2-[2-[2-[2-[2-(2-Aminoethoxy)ethoxy]ethoxy]ethoxy]ethoxy]ethoxy]ethoxy]ethoxy]ethoxy]ethoxy]ethoxy]ethoxy]propanoic acid
  SITE 20: note = 3-[2-[2-[2-[2-[2-[2-[2-[2-[2-[2-[2-(2-Aminoethoxy)ethoxy]ethoxy]ethoxy]ethoxy]ethoxy]ethoxy]ethoxy]ethoxy]ethoxy]ethoxy]ethoxy]propanoic acid
  SITE 1..12: note = Thiol group of cysteine is linked to N-terminal end of 3-(2-Naphthyl)-L-alanine via -CH2-CO-
  SITE 21: note = Amidation of C-terminal carboxyl group
  SITE 21: note = Lysine side chain is modified with maleimide
XRSGXNWXRWXCGGGGDXDXK

SEQ ID NO: 49 - protein, 21 aa, synthetic construct
  REGION 1..21: note = Peptide-49
  SITE 1: note = 3-(2-Naphthyl)-L-alanine
  SITE 5: note = (2S)-2-Amino-4-guanidino-butanoic acid
  SITE 8: note = Nle
  SITE 11: note = L-Alpha-cyclohexylglycine
  REGION 18..19: note = 3-[2-[2-[2-[2-[2-[2-[2-[2-[2-[2-[2-(2-Aminoethoxy)ethoxy]ethoxy]ethoxy]ethoxy]ethoxy]ethoxy]ethoxy]ethoxy]ethoxy]ethoxy]ethoxy]propanoic acid
  SITE 1..12: note = Thiol group of cysteine is linked to N-terminal end of 3-(2-Naphthyl)-L-alanine via -CH2-CO-
  SITE 21: note = Amidation of C-terminal carboxyl group
  SITE 21: note = Lysine side chain is modified with maleimide
XRSGXNWXRWXCGGGGDXXDK

SEQ ID NO: 50 - protein, 21 aa, synthetic construct
  REGION 1..21: note = Peptide-50
  SITE 1: note = 3-(2-Naphthyl)-L-alanine
  SITE 5: note = (2S)-2-Amino-4-guanidino-butanoic acid
  SITE 8: note = Nle
  SITE 11: note = L-Alpha-cyclohexylglycine
  SITE 17: note = 3-[2-[2-[2-[2-[2-[2-[2-[2-[2-[2-[2-(2-Aminoethoxy)ethoxy]ethoxy]ethoxy]ethoxy]ethoxy]ethoxy]ethoxy]ethoxy]ethoxy]ethoxy]ethoxy]propanoic acid
  SITE 19: note = 3-[2-[2-[2-[2-[2-[2-[2-[2-[2-[2-[2-(2-Aminoethoxy)ethoxy]ethoxy]ethoxy]ethoxy]ethoxy]ethoxy]ethoxy]ethoxy]ethoxy]ethoxy]ethoxy]propanoic acid
  SITE 1..12: note = Thiol group of cysteine is linked to N-terminal end of 3-(2-Naphthyl)-L-alanine via -CH2-CO-
  SITE 21: note = Amidation of C-terminal carboxyl group
  SITE 21: note = Lysine side chain is modified with maleimide
XRSGXNWXRWXCGGGGXDXDK

SEQ ID NO: 51 - protein, 22 aa, synthetic construct
  REGION 1..22: note = Peptide-51
  SITE 1: note = 3-(2-Naphthyl)-L-alanine
  SITE 5: note = (2S)-2-Amino-4-guanidino-butanoic acid
  SITE 8: note = Nle
  SITE 11: note = L-Alpha-cyclohexylglycine
  SITE 19: note = (2S)-6-amino-2-[[2-[2-[2-[2-[2-[2-[2-[2-[2-[2-(2-methoxyethoxy)ethoxy]ethoxy]ethoxy]ethoxy]ethoxy]ethoxy]ethoxy]ethoxy]ethoxy]acetyl]amino]hexanoic acid
  REGION 20..21: note = 3-[2-[2-[2-[2-[2-[2-[2-[2-[2-[2-[2-(2-Aminoethoxy)ethoxy]ethoxy]ethoxy]ethoxy]ethoxy]ethoxy]ethoxy]ethoxy]ethoxy]ethoxy]ethoxy]propanoic acid
  SITE 1..12: note = Thiol group of cysteine is linked to N-terminal end of 3-(2-Naphthyl)-L-alanine via -CH2-CO-
  SITE 22: note = Amidation of C-terminal carboxyl group
  SITE 22: note = Lysine side chain is modified with maleimide
XRSGXNWXRWXCGGGGDDXXXK

SEQ ID NO: 52 - protein, 22 aa, synthetic construct
  REGION 1..22: note = Peptide-52
  SITE 1: note = 3-(2-Naphthyl)-L-alanine
  SITE 5: note = (2S)-2-Amino-4-guanidino-butanoic acid
  SITE 8: note = Nle
  SITE 11: note = L-Alpha-cyclohexylglycine
  SITE 19: note = 3-[2-[2-[2-[2-[2-[2-[2-[2-[2-[2-[2-(2-Aminoethoxy)ethoxy]ethoxy]ethoxy]ethoxy]ethoxy]ethoxy]ethoxy]ethoxy]ethoxy]ethoxy]ethoxy]propanoic acid
  SITE 20: note = (2S)-6-amino-2-[[2-[2-[2-[2-[2-[2-[2-[2-[2-[2-(2-methoxyethoxy)ethoxy]ethoxy]ethoxy]ethoxy]ethoxy]ethoxy]ethoxy]ethoxy]ethoxy]acetyl]amino]hexanoic acid
  SITE 21: note = 3-[2-[2-[2-[2-[2-[2-[2-[2-[2-[2-[2-(2-Aminoethoxy)ethoxy]ethoxy]ethoxy]ethoxy]ethoxy]ethoxy]ethoxy]ethoxy]ethoxy]ethoxy]ethoxy]propanoic acid
  SITE 1..12: note = Thiol group of cysteine is linked to N-terminal end of 3-(2-Naphthyl)-L-alanine via -CH2-CO-
  SITE 22: note = Amidation of C-terminal carboxyl group
  SITE 22: note = Lysine side chain is modified with maleimide
XRSGXNWXRWXCGGGGDDXXXK

SEQ ID NO: 53 - protein, 22 aa, synthetic construct
  REGION 1..22: note = Peptide-53
  SITE 1: note = 3-(2-Naphthyl)-L-alanine
  SITE 5: note = (2S)-2-Amino-4-guanidino-butanoic acid
  SITE 8: note = Nle
  SITE 11: note = L-Alpha-cyclohexylglycine
  REGION 19..20: note = 3-[2-[2-[2-[2-[2-[2-[2-[2-[2-[2-[2-(2-Aminoethoxy)ethoxy]ethoxy]ethoxy]ethoxy]ethoxy]ethoxy]ethoxy]ethoxy]ethoxy]ethoxy]ethoxy]propanoic acid
  SITE 21: note = (2S)-6-amino-2-[[2-[2-[2-[2-[2-[2-[2-[2-[2-[2-(2-methoxyethoxy)ethoxy]ethoxy]ethoxy]ethoxy]ethoxy]ethoxy]ethoxy]ethoxy]ethoxy]acetyl]amino]hexanoic acid
  SITE 1..12: note = Thiol group of cysteine is linked to N-terminal end of 3-(2-Naphthyl)-L-alanine via -CH2-CO-
  SITE 22: note = Amidation of C-terminal carboxyl group
  SITE 22: note = Lysine side chain is modified with maleimide
XRSGXNWXRWXCGGGGDDXXXK

SEQ ID NO: 54 - protein, 22 aa, synthetic construct
  REGION 1..22: note = Peptide-54
  SITE 1: note = 3-(2-Naphthyl)-L-alanine
  SITE 5: note = (2S)-2-Amino-4-guanidino-butanoic acid
  SITE 11: note = L-Cyclopentylglycine
  SITE 19: note = (2S)-6-amino-2-[[2-[2-[2-[2-[2-[2-[2-[2-[2-[2-(2-methoxyethoxy)ethoxy]ethoxy]ethoxy]ethoxy]ethoxy]ethoxy]ethoxy]ethoxy]ethoxy]acetyl]amino]hexanoic acid
  REGION 20..21: note = 3-[2-[2-[2-[2-[2-[2-[2-[2-[2-[2-[2-(2-Aminoethoxy)ethoxy]ethoxy]ethoxy]ethoxy]ethoxy]ethoxy]ethoxy]ethoxy]ethoxy]ethoxy]ethoxy]propanoic acid
  SITE 1..12: note = Thiol group of cysteine is linked to N-terminal end of 3-(2-Naphthyl)-L-alanine via -CH2-CO-
  SITE 22: note = Amidation of C-terminal carboxyl group
  SITE 22: note = Lysine side chain is modified with maleimide
XRSGXNWVRWXCGGGGDDXXXK

SEQ ID NO: 55 - protein, 22 aa, synthetic construct
  REGION 1..22: note = Peptide-55
  SITE 1: note = 3-(2-Naphthyl)-L-alanine
  SITE 5: note = (2S)-2-Amino-4-guanidino-butanoic acid
  SITE 11: note = L-Cyclopentylglycine
  SITE 19: note = 3-[2-[2-[2-[2-[2-[2-[2-[2-[2-[2-[2-(2-Aminoethoxy)ethoxy]ethoxy]ethoxy]ethoxy]ethoxy]ethoxy]ethoxy]ethoxy]ethoxy]ethoxy]ethoxy]propanoic acid
  SITE 20: note = (2S)-6-amino-2-[[2-[2-[2-[2-[2-[2-[2-[2-[2-[2-(2-methoxyethoxy)ethoxy]ethoxy]ethoxy]ethoxy]ethoxy]ethoxy]ethoxy]ethoxy]ethoxy]acetyl]amino]hexanoic acid
  SITE 21: note = 3-[2-[2-[2-[2-[2-[2-[2-[2-[2-[2-[2-(2-Aminoethoxy)ethoxy]ethoxy]ethoxy]ethoxy]ethoxy]ethoxy]ethoxy]ethoxy]ethoxy]ethoxy]ethoxy]propanoic acid
  SITE 1..12: note = Thiol group of cysteine is linked to N-terminal end of 3-(2-Naphthyl)-L-alanine via -CH2-CO-
  SITE 22: note = Amidation of C-terminal carboxyl group
  SITE 22: note = Lysine side chain is modified with maleimide
XRSGXNWVRWXCGGGGDDXXXK

SEQ ID NO: 56 - protein, 22 aa, synthetic construct
  REGION 1..22: note = Peptide-56
  SITE 1: note = 3-(2-Naphthyl)-L-alanine
  SITE 5: note = (2S)-2-Amino-4-guanidino-butanoic acid
  SITE 11: note = L-Cyclopentylglycine
  REGION 19..20: note = 3-[2-[2-[2-[2-[2-[2-[2-[2-[2-[2-[2-(2-Aminoethoxy)ethoxy]ethoxy]ethoxy]ethoxy]ethoxy]ethoxy]ethoxy]ethoxy]ethoxy]ethoxy]ethoxy]propanoic acid
  SITE 21: note = (2S)-6-amino-2-[[2-[2-[2-[2-[2-[2-[2-[2-[2-[2-(2-methoxyethoxy)ethoxy]ethoxy]ethoxy]ethoxy]ethoxy]ethoxy]ethoxy]ethoxy]ethoxy]acetyl]amino]hexanoic acid
  SITE 1..12: note = Thiol group of cysteine is linked to N-terminal end of 3-(2-Naphthyl)-L-alanine via -CH2-CO-
  SITE 22: note = Amidation of C-terminal carboxyl group
  SITE 22: note = Lysine side chain is modified with maleimide
XRSGXNWVRWXCGGGGDDXXXK

SEQ ID NO: 57 - protein, 21 aa, synthetic construct
  REGION 1..21: note = Peptide-57
  SITE 1: note = 3-(2-Naphthyl)-L-alanine
  SITE 5: note = (2S)-2-Amino-4-guanidino-butanoic acid
  SITE 11: note = L-Cyclopentylglycine
  SITE 18: note = 3-[2-[2-[2-[2-[2-(2-Aminoethoxy)ethoxy]ethoxy]ethoxy]ethoxy]ethoxy]propanoic acid
  SITE 20: note = 3-[2-[2-[2-[2-[2-(2-Aminoethoxy)ethoxy]ethoxy]ethoxy]ethoxy]ethoxy]propanoic acid
  SITE 1..12: note = Thiol group of cysteine is linked to N-terminal end of 3-(2-Naphthyl)-L-alanine via -CH2-CO-
  SITE 21: note = Amidation of C-terminal carboxyl group
  SITE 21: note = Lysine side chain is modified with maleimide
XRSGXNWVRWXCGGGGDXDXK

SEQ ID NO: 58 - protein, 21 aa, synthetic construct
  REGION 1..21: note = Peptide-58
  SITE 1: note = 3-(2-Naphthyl)-L-alanine
  SITE 5: note = (2S)-2-Amino-4-guanidino-butanoic acid
  SITE 11: note = L-Cyclopentylglycine
  SITE 17: note = 3-[2-[2-[2-[2-[2-(2-Aminoethoxy)ethoxy]ethoxy]ethoxy]ethoxy]ethoxy]propanoic acid
  SITE 20: note = 3-[2-[2-[2-[2-[2-(2-Aminoethoxy)ethoxy]ethoxy]ethoxy]ethoxy]ethoxy]propanoic acid
  SITE 1..12: note = Thiol group of cysteine is linked to N-terminal end of 3-(2-Naphthyl)-L-alanine via -CH2-CO-
  SITE 21: note = Amidation of C-terminal carboxyl group
  SITE 21: note = Lysine side chain is modified with maleimide
XRSGXNWVRWXCGGGGXDDXK

SEQ ID NO: 59 - protein, 21 aa, synthetic construct
  REGION 1..21: note = Peptide-59
  SITE 1: note = 3-(2-Naphthyl)-L-alanine
  SITE 5: note = (2S)-2-Amino-4-guanidino-butanoic acid
  SITE 11: note = L-Cyclopentylglycine
  SITE 17: note = 3-[2-[2-[2-[2-[2-(2-Aminoethoxy)ethoxy]ethoxy]ethoxy]ethoxy]ethoxy]propanoic acid
  SITE 19: note = 3-[2-[2-[2-[2-[2-(2-Aminoethoxy)ethoxy]ethoxy]ethoxy]ethoxy]ethoxy]propanoic acid
  SITE 1..12: note = Thiol group of cysteine is linked to N-terminal end of 3-(2-Naphthyl)-L-alanine via -CH2-CO-
  SITE 21: note = Amidation of C-terminal carboxyl group
  SITE 21: note = Lysine side chain is modified with maleimide
XRSGXNWVRWXCGGGGXDXDK

SEQ ID NO: 60 - protein, 22 aa, synthetic construct
  REGION 1..22: note = Peptide-60
  SITE 1: note = 3-(2-Naphthyl)-L-alanine
  SITE 5: note = (2S)-2-Amino-4-guanidino-butanoic acid
  SITE 8: note = Nle
  SITE 11: note = L-Alpha-cyclohexylglycine
  SITE 19: note = (2R,4S,5R,6R)-5-acetamido-2-[[(2R,3R,4S,5R,6S)-6-[(2R,3S,4R,5R,6S)-5-acetamido-6-[(2S,3S,4S,5S,6R)-2-[[(2R,3R,4S,5S,6S)-6-[(2R,3S,4R,5R,6S)-5-acetamido-6-[(2R,3S,4R,5R,6R)-5-acetamido-6-[2-[[(5S)-5-amino-5-carboxy-pentyl]amino]-2-oxo-ethoxy]-4-hydroxy-2-(hydroxymethyl)tetrahydropyran-3-yl]oxy-4-hydroxy-2-(hydroxymethyl)tetrahydropyran-3-yl]oxy-4-[(2R,3S,4S,5S,6R)-3-[(2S,3R,4R,5S,6R)-3-acetamido-5-[(2S,3R,4S,5R,6R)-6-[[(2R,4S,5R,6R)-5-acetamido-2-carboxy-4-hydroxy-6-[(1R,2R)-1,2,3-trihydroxypropyl]tetrahydropyran-2-yl]oxymethyl]-3,4,5-trihydroxy-tetrahydropyran-2-yl]oxy-4-hydroxy-6-(hydroxymethyl)tetrahydropyran-2-yl]oxy-4,5-dihydroxy-6-(hydroxymethyl)tetrahydropyran-2-yl]oxy-3,5-dihydroxy-tetrahydropyran-2-yl]methoxy]-4,5-dihydroxy-6-(hydroxymethyl)tetrahydropyran-3-yl]oxy-4-hydroxy-2-(hydroxymethyl)tetrahydropyran-3-yl]oxy-3,4,5-trihydroxy-tetrahydropyran-2-yl]methoxy]-4-hydroxy-6-[(1R,2R)-1,2,3-trihydroxypropyl]tetrahydropyran-2-carboxylic acid
  REGION 20..21: note = 3-[2-[2-[2-[2-[2-[2-[2-[2-[2-[2-[2-(2-Aminoethoxy)ethoxy]ethoxy]ethoxy]ethoxy]ethoxy]ethoxy]ethoxy]ethoxy]ethoxy]ethoxy]ethoxy]propanoic acid
  SITE 1..12: note = Thiol group of cysteine is linked to N-terminal end of 3-(2-Naphthyl)-L-alanine via -CH2-CO-
  SITE 22: note = Amidation of C-terminal carboxyl group
  SITE 22: note = Lysine side chain is modified with maleimide
XRSGXNWXRWXCGGGGDDXXXK

SEQ ID NO: 61 - protein, 22 aa, synthetic construct
  REGION 1..22: note = Peptide-61
  SITE 1: note = 3-(2-Naphthyl)-L-alanine
  SITE 5: note = (2S)-2-Amino-4-guanidino-butanoic acid
  SITE 8: note = Nle
  SITE 11: note = L-Alpha-cyclohexylglycine
  SITE 19: note = 3-[2-[2-[2-[2-[2-[2-[2-[2-[2-[2-[2-(2-Aminoethoxy)ethoxy]ethoxy]ethoxy]ethoxy]ethoxy]ethoxy]ethoxy]ethoxy]ethoxy]ethoxy]ethoxy]propanoic acid
  SITE 20: note = (2R,4S,5R,6R)-5-acetamido-2-[[(2R,3R,4S,5R,6S)-6-[(2R,3S,4R,5R,6S)-5-acetamido-6-[(2S,3S,4S,5S,6R)-2-[[(2R,3R,4S,5S,6S)-6-[(2R,3S,4R,5R,6S)-5-acetamido-6-[(2R,3S,4R,5R,6R)-5-acetamido-6-[2-[[(5S)-5-amino-5-carboxy-pentyl]amino]-2-oxo-ethoxy]-4-hydroxy-2-(hydroxymethyl)tetrahydropyran-3-yl]oxy-4-hydroxy-2-(hydroxymethyl)tetrahydropyran-3-yl]oxy-4-[(2R,3S,4S,5S,6R)-3-[(2S,3R,4R,5S,6R)-3-acetamido-5-[(2S,3R,4S,5R,6R)-6-[[(2R,4S,5R,6R)-5-acetamido-2-carboxy-4-hydroxy-6-[(1R,2R)-1,2,3-trihydroxypropyl]tetrahydropyran-2-yl]oxymethyl]-3,4,5-trihydroxy-tetrahydropyran-2-yl]oxy-4-hydroxy-6-(hydroxymethyl)tetrahydropyran-2-yl]oxy-4,5-dihydroxy-6-(hydroxymethyl)tetrahydropyran-2-yl]oxy-3,5-dihydroxy-tetrahydropyran-2-yl]methoxy]-4,5-dihydroxy-6-(hydroxymethyl)tetrahydropyran-3-yl]oxy-4-hydroxy-2-(hydroxymethyl)tetrahydropyran-3-yl]oxy-3,4,5-trihydroxy-tetrahydropyran-2-yl]methoxy]-4-hydroxy-6-[(1R,2R)-1,2,3-trihydroxypropyl]tetrahydropyran-2-carboxylic acid
  SITE 21: note = 3-[2-[2-[2-[2-[2-[2-[2-[2-[2-[2-[2-(2-Aminoethoxy)ethoxy]ethoxy]ethoxy]ethoxy]ethoxy]ethoxy]ethoxy]ethoxy]ethoxy]ethoxy]ethoxy]propanoic acid
  SITE 1..12: note = Thiol group of cysteine is linked to N-terminal end of 3-(2-Naphthyl)-L-alanine via -CH2-CO-
  SITE 22: note = Amidation of C-terminal carboxyl group
  SITE 22: note = Lysine side chain is modified with maleimide
XRSGXNWXRWXCGGGGDDXXXK

SEQ ID NO: 62 - protein, 20 aa, synthetic construct
  REGION 1..20: note = Peptide-62
  SITE 1: note = 3-(2-Naphthyl)-L-alanine
  SITE 5: note = (2S)-2-Amino-4-guanidino-butanoic acid
  SITE 8: note = Nle
  SITE 11: note = L-Alpha-cyclohexylglycine
  SITE 17: note = (2R,4S,5R,6R)-5-acetamido-2-[[(2R,3R,4S,5R,6S)-6-[(2R,3S,4R,5R,6S)-5-acetamido-6-[(2S,3S,4S,5S,6R)-2-[[(2R,3R,4S,5S,6S)-6-[(2R,3S,4R,5R,6S)-5-acetamido-6-[(2R,3S,4R,5R,6R)-5-acetamido-6-[2-[[(5S)-5-amino-5-carboxy-pentyl]amino]-2-oxo-ethoxy]-4-hydroxy-2-(hydroxymethyl)tetrahydropyran-3-yl]oxy-4-hydroxy-2-(hydroxymethyl)tetrahydropyran-3-yl]oxy-4-[(2R,3S,4S,5S,6R)-3-[(2S,3R,4R,5S,6R)-3-acetamido-5-[(2S,3R,4S,5R,6R)-6-[[(2R,4S,5R,6R)-5-acetamido-2-carboxy-4-hydroxy-6-[(1R,2R)-1,2,3-trihydroxypropyl]tetrahydropyran-2-yl]oxymethyl]-3,4,5-trihydroxy-tetrahydropyran-2-yl]oxy-4-hydroxy-6-(hydroxymethyl)tetrahydropyran-2-yl]oxy-4,5-dihydroxy-6-(hydroxymethyl)tetrahydropyran-2-yl]oxy-3,5-dihydroxy-tetrahydropyran-2-yl]methoxy]-4,5-dihydroxy-6-(hydroxymethyl)tetrahydropyran-3-yl]oxy-4-hydroxy-2-(hydroxymethyl)tetrahydropyran-3-yl]oxy-3,4,5-trihydroxy-tetrahydropyran-2-yl]methoxy]-4-hydroxy-6-[(1R,2R)-1,2,3-trihydroxypropyl]tetrahydropyran-2-carboxylic acid
  REGION 18..19: note = 3-[2-[2-[2-[2-[2-[2-[2-[2-[2-[2-[2-(2-Aminoethoxy)ethoxy]ethoxy]ethoxy]ethoxy]ethoxy]ethoxy]ethoxy]ethoxy]ethoxy]ethoxy]ethoxy]propanoic acid
  SITE 1..12: note = Thiol group of cysteine is linked to N-terminal end of 3-(2-Naphthyl)-L-alanine via -CH2-CO-
  SITE 20: note = Amidation of C-terminal carboxyl group
  SITE 20: note = Lysine side chain is modified with maleimide
XRSGXNWXRWXCGGGGXXXK

SEQ ID NO: 63 - protein, 20 aa, synthetic construct
  REGION 1..20: note = Peptide-63
  SITE 1: note = 3-(2-Naphthyl)-L-alanine
  SITE 5: note = (2S)-2-Amino-4-guanidino-butanoic acid
  SITE 8: note = Nle
  SITE 11: note = L-Alpha-cyclohexylglycine
  SITE 17: note = 3-[2-[2-[2-[2-[2-[2-[2-[2-[2-[2-[2-(2-Aminoethoxy)ethoxy]ethoxy]ethoxy]ethoxy]ethoxy]ethoxy]ethoxy]ethoxy]ethoxy]ethoxy]ethoxy]propanoic acid
  SITE 18: note = (2R,4S,5R,6R)-5-acetamido-2-[[(2R,3R,4S,5R,6S)-6-[(2R,3S,4R,5R,6S)-5-acetamido-6-[(2S,3S,4S,5S,6R)-2-[[(2R,3R,4S,5S,6S)-6-[(2R,3S,4R,5R,6S)-5-acetamido-6-[(2R,3S,4R,5R,6R)-5-acetamido-6-[2-[[(5S)-5-amino-5-carboxy-pentyl]amino]-2-oxo-ethoxy]-4-hydroxy-2-(hydroxymethyl)tetrahydropyran-3-yl]oxy-4-hydroxy-2-(hydroxymethyl)tetrahydropyran-3-yl]oxy-4-[(2R,3S,4S,5S,6R)-3-[(2S,3R,4R,5S,6R)-3-acetamido-5-[(2S,3R,4S,5R,6R)-6-[[(2R,4S,5R,6R)-5-acetamido-2-carboxy-4-hydroxy-6-[(1R,2R)-1,2,3-trihydroxypropyl]tetrahydropyran-2-yl]oxymethyl]-3,4,5-trihydroxy-tetrahydropyran-2-yl]oxy-4-hydroxy-6-(hydroxymethyl)tetrahydropyran-2-yl]oxy-4,5-dihydroxy-6-(hydroxymethyl)tetrahydropyran-2-yl]oxy-3,5-dihydroxy-tetrahydropyran-2-yl]methoxy]-4,5-dihydroxy-6-(hydroxymethyl)tetrahydropyran-3-yl]oxy-4-hydroxy-2-(hydroxymethyl)tetrahydropyran-3-yl]oxy-3,4,5-trihydroxy-tetrahydropyran-2-yl]methoxy]-4-hydroxy-6-[(1R,2R)-1,2,3-trihydroxypropyl]tetrahydropyran-2-carboxylic acid
  SITE 19: note = 3-[2-[2-[2-[2-[2-[2-[2-[2-[2-[2-[2-(2-Aminoethoxy)ethoxy]ethoxy]ethoxy]ethoxy]ethoxy]ethoxy]ethoxy]ethoxy]ethoxy]ethoxy]ethoxy]propanoic acid
  SITE 1..12: note = Thiol group of cysteine is linked to N-terminal end of 3-(2-Naphthyl)-L-alanine via -CH2-CO-
  SITE 20: note = Amidation of C-terminal carboxyl group
  SITE 20: note = Lysine side chain is modified with maleimide
XRSGXNWXRWXCGGGGXXXK

SEQ ID NO: 64 - protein, 20 aa, synthetic construct
  REGION 1..20: note = Peptide-64
  SITE 1: note = 3-(2-Naphthyl)-L-alanine
  SITE 5: note = (2S)-2-Amino-4-guanidino-butanoic acid
  SITE 8: note = Nle
  SITE 11: note = L-Alpha-cyclohexylglycine
  REGION 17..18: note = 3-[2-[2-[2-[2-[2-[2-[2-[2-[2-[2-[2-(2-Aminoethoxy)ethoxy]ethoxy]ethoxy]ethoxy]ethoxy]ethoxy]ethoxy]ethoxy]ethoxy]ethoxy]ethoxy]propanoic acid
  SITE 19: note = (2R,4S,5R,6R)-5-acetamido-2-[[(2R,3R,4S,5R,6S)-6-[(2R,3S,4R,5R,6S)-5-acetamido-6-[(2S,3S,4S,5S,6R)-2-[[(2R,3R,4S,5S,6S)-6-[(2R,3S,4R,5R,6S)-5-acetamido-6-[(2R,3S,4R,5R,6R)-5-acetamido-6-[2-[[(5S)-5-amino-5-carboxy-pentyl]amino]-2-oxo-ethoxy]-4-hydroxy-2-(hydroxymethyl)tetrahydropyran-3-yl]oxy-4-hydroxy-2-(hydroxymethyl)tetrahydropyran-3-yl]oxy-4-[(2R,3S,4S,5S,6R)-3-[(2S,3R,4R,5S,6R)-3-acetamido-5-[(2S,3R,4S,5R,6R)-6-[[(2R,4S,5R,6R)-5-acetamido-2-carboxy-4-hydroxy-6-[(1R,2R)-1,2,3-trihydroxypropyl]tetrahydropyran-2-yl]oxymethyl]-3,4,5-trihydroxy-tetrahydropyran-2-yl]oxy-4-hydroxy-6-(hydroxymethyl)tetrahydropyran-2-yl]oxy-4,5-dihydroxy-6-(hydroxymethyl)tetrahydropyran-2-yl]oxy-3,5-dihydroxy-tetrahydropyran-2-yl]methoxy]-4,5-dihydroxy-6-(hydroxymethyl)tetrahydropyran-3-yl]oxy-4-hydroxy-2-(hydroxymethyl)tetrahydropyran-3-yl]oxy-3,4,5-trihydroxy-tetrahydropyran-2-yl]methoxy]-4-hydroxy-6-[(1R,2R)-1,2,3-trihydroxypropyl]tetrahydropyran-2-carboxylic acid
  SITE 1..12: note = Thiol group of cysteine is linked to N-terminal end of 3-(2-Naphthyl)-L-alanine via -CH2-CO-
  SITE 20: note = Amidation of C-terminal carboxyl group
  SITE 20: note = Lysine side chain is modified with maleimide
XRSGXNWXRWXCGGGGXXXK

SEQ ID NO: 65 - protein, 22 aa, synthetic construct
  REGION 1..22: note = Peptide-65
  SITE 1: note = 3-(2-Naphthyl)-L-alanine
  SITE 5: note = (2S)-2-Amino-4-guanidino-butanoic acid
  SITE 11: note = L-Cyclopentylglycine
  SITE 19: note = (2R,4S,5R,6R)-5-acetamido-2-[[(2R,3R,4S,5R,6S)-6-[(2R,3S,4R,5R,6S)-5-acetamido-6-[(2S,3S,4S,5S,6R)-2-[[(2R,3R,4S,5S,6S)-6-[(2R,3S,4R,5R,6S)-5-acetamido-6-[(2R,3S,4R,5R,6R)-5-acetamido-6-[2-[[(5S)-5-amino-5-carboxy-pentyl]amino]-2-oxo-ethoxy]-4-hydroxy-2-(hydroxymethyl)tetrahydropyran-3-yl]oxy-4-hydroxy-2-(hydroxymethyl)tetrahydropyran-3-yl]oxy-4-[(2R,3S,4S,5S,6R)-3-[(2S,3R,4R,5S,6R)-3-acetamido-5-[(2S,3R,4S,5R,6R)-6-[[(2R,4S,5R,6R)-5-acetamido-2-carboxy-4-hydroxy-6-[(1R,2R)-1,2,3-trihydroxypropyl]tetrahydropyran-2-yl]oxymethyl]-3,4,5-trihydroxy-tetrahydropyran-2-yl]oxy-4-hydroxy-6-(hydroxymethyl)tetrahydropyran-2-yl]oxy-4,5-dihydroxy-6-(hydroxymethyl)tetrahydropyran-2-yl]oxy-3,5-dihydroxy-tetrahydropyran-2-yl]methoxy]-4,5-dihydroxy-6-(hydroxymethyl)tetrahydropyran-3-yl]oxy-4-hydroxy-2-(hydroxymethyl)tetrahydropyran-3-yl]oxy-3,4,5-trihydroxy-tetrahydropyran-2-yl]methoxy]-4-hydroxy-6-[(1R,2R)-1,2,3-trihydroxypropyl]tetrahydropyran-2-carboxylic acid
  REGION 20..21: note = 3-[2-[2-[2-[2-[2-[2-[2-[2-[2-[2-[2-(2-Aminoethoxy)ethoxy]ethoxy]ethoxy]ethoxy]ethoxy]ethoxy]ethoxy]ethoxy]ethoxy]ethoxy]ethoxy]propanoic acid
  SITE 1..12: note = Thiol group of cysteine is linked to N-terminal end of 3-(2-Naphthyl)-L-alanine via -CH2-CO-
  SITE 22: note = Amidation of C-terminal carboxyl group
  SITE 22: note = Lysine side chain is modified with maleimide
XRSGXNWVRWXCGGGGDDXXXK

SEQ ID NO: 66 - protein, 22 aa, synthetic construct
  REGION 1..22: note = Peptide-66
  SITE 1: note = 3-(2-Naphthyl)-L-alanine
  SITE 5: note = (2S)-2-Amino-4-guanidino-butanoic acid
  SITE 11: note = L-Cyclopentylglycine
  SITE 19: note = 3-[2-[2-[2-[2-[2-[2-[2-[2-[2-[2-[2-(2-Aminoethoxy)ethoxy]ethoxy]ethoxy]ethoxy]ethoxy]ethoxy]ethoxy]ethoxy]ethoxy]ethoxy]ethoxy]propanoic acid
  SITE 20: note = (2R,4S,5R,6R)-5-acetamido-2-[[(2R,3R,4S,5R,6S)-6-[(2R,3S,4R,5R,6S)-5-acetamido-6-[(2S,3S,4S,5S,6R)-2-[[(2R,3R,4S,5S,6S)-6-[(2R,3S,4R,5R,6S)-5-acetamido-6-[(2R,3S,4R,5R,6R)-5-acetamido-6-[2-[[(5S)-5-amino-5-carboxy-pentyl]amino]-2-oxo-ethoxy]-4-hydroxy-2-(hydroxymethyl)tetrahydropyran-3-yl]oxy-4-hydroxy-2-(hydroxymethyl)tetrahydropyran-3-yl]oxy-4-[(2R,3S,4S,5S,6R)-3-[(2S,3R,4R,5S,6R)-3-acetamido-5-[(2S,3R,4S,5R,6R)-6-[[(2R,4S,5R,6R)-5-acetamido-2-carboxy-4-hydroxy-6-[(1R,2R)-1,2,3-trihydroxypropyl]tetrahydropyran-2-yl]oxymethyl]-3,4,5-trihydroxy-tetrahydropyran-2-yl]oxy-4-hydroxy-6-(hydroxymethyl)tetrahydropyran-2-yl]oxy-4,5-dihydroxy-6-(hydroxymethyl)tetrahydropyran-2-yl]oxy-3,5-dihydroxy-tetrahydropyran-2-yl]methoxy]-4,5-dihydroxy-6-(hydroxymethyl)tetrahydropyran-3-yl]oxy-4-hydroxy-2-(hydroxymethyl)tetrahydropyran-3-yl]oxy-3,4,5-trihydroxy-tetrahydropyran-2-yl]methoxy]-4-hydroxy-6-[(1R,2R)-1,2,3-trihydroxypropyl]tetrahydropyran-2-carboxylic acid
  SITE 21: note = 3-[2-[2-[2-[2-[2-[2-[2-[2-[2-[2-[2-(2-Aminoethoxy)ethoxy]ethoxy]ethoxy]ethoxy]ethoxy]ethoxy]ethoxy]ethoxy]ethoxy]ethoxy]ethoxy]propanoic acid
  SITE 1..12: note = Thiol group of cysteine is linked to N-terminal end of 3-(2-Naphthyl)-L-alanine via -CH2-CO-
  SITE 22: note = Amidation of C-terminal carboxyl group
  SITE 22: note = Lysine side chain is modified with maleimide
XRSGXNWVRWXCGGGGDDXXXK

SEQ ID NO: 67 - protein, 22 aa, synthetic construct
  REGION 1..22: note = Peptide-67
  SITE 1: note = 3-(2-Naphthyl)-L-alanine
  SITE 5: note = (2S)-2-Amino-4-guanidino-butanoic acid
  SITE 11: note = L-Cyclopentylglycine
  REGION 19..20: note = 3-[2-[2-[2-[2-[2-[2-[2-[2-[2-[2-[2-(2-Aminoethoxy)ethoxy]ethoxy]ethoxy]ethoxy]ethoxy]ethoxy]ethoxy]ethoxy]ethoxy]ethoxy]ethoxy]propanoic acid
  SITE 21: note = (2R,4S,5R,6R)-5-acetamido-2-[[(2R,3R,4S,5R,6S)-6-[(2R,3S,4R,5R,6S)-5-acetamido-6-[(2S,3S,4S,5S,6R)-2-[[(2R,3R,4S,5S,6S)-6-[(2R,3S,4R,5R,6S)-5-acetamido-6-[(2R,3S,4R,5R,6R)-5-acetamido-6-[2-[[(5S)-5-amino-5-carboxy-pentyl]amino]-2-oxo-ethoxy]-4-hydroxy-2-(hydroxymethyl)tetrahydropyran-3-yl]oxy-4-hydroxy-2-(hydroxymethyl)tetrahydropyran-3-yl]oxy-4-[(2R,3S,4S,5S,6R)-3-[(2S,3R,4R,5S,6R)-3-acetamido-5-[(2S,3R,4S,5R,6R)-6-[[(2R,4S,5R,6R)-5-acetamido-2-carboxy-4-hydroxy-6-[(1R,2R)-1,2,3-trihydroxypropyl]tetrahydropyran-2-yl]oxymethyl]-3,4,5-trihydroxy-tetrahydropyran-2-yl]oxy-4-hydroxy-6-(hydroxymethyl)tetrahydropyran-2-yl]oxy-4,5-dihydroxy-6-(hydroxymethyl)tetrahydropyran-2-yl]oxy-3,5-dihydroxy-tetrahydropyran-2-yl]methoxy]-4,5-dihydroxy-6-(hydroxymethyl)tetrahydropyran-3-yl]oxy-4-hydroxy-2-(hydroxymethyl)tetrahydropyran-3-yl]oxy-3,4,5-trihydroxy-tetrahydropyran-2-yl]methoxy]-4-hydroxy-6-[(1R,2R)-1,2,3-trihydroxypropyl]tetrahydropyran-2-carboxylic acid
  SITE 1..12: note = Thiol group of cysteine is linked to N-terminal end of 3-(2-Naphthyl)-L-alanine via -CH2-CO-
  SITE 22: note = Amidation of C-terminal carboxyl group
  SITE 22: note = Lysine side chain is modified with maleimide
XRSGXNWVRWXCGGGGDDXXXK

SEQ ID NO: 68 - protein, 20 aa, synthetic construct
  REGION 1..20: note = Peptide-68
  SITE 1: note = 3-(2-Naphthyl)-L-alanine
  SITE 5: note = (2S)-2-Amino-4-guanidino-butanoic acid
  SITE 11: note = L-Cyclopentylglycine
  SITE 17: note = (2R,4S,5R,6R)-5-acetamido-2-[[(2R,3R,4S,5R,6S)-6-[(2R,3S,4R,5R,6S)-5-acetamido-6-[(2S,3S,4S,5S,6R)-2-[[(2R,3R,4S,5S,6S)-6-[(2R,3S,4R,5R,6S)-5-acetamido-6-[(2R,3S,4R,5R,6R)-5-acetamido-6-[2-[[(5S)-5-amino-5-carboxy-pentyl]amino]-2-oxo-ethoxy]-4-hydroxy-2-(hydroxymethyl)tetrahydropyran-3-yl]oxy-4-hydroxy-2-(hydroxymethyl)tetrahydropyran-3-yl]oxy-4-[(2R,3S,4S,5S,6R)-3-[(2S,3R,4R,5S,6R)-3-acetamido-5-[(2S,3R,4S,5R,6R)-6-[[(2R,4S,5R,6R)-5-acetamido-2-carboxy-4-hydroxy-6-[(1R,2R)-1,2,3-trihydroxypropyl]tetrahydropyran-2-yl]oxymethyl]-3,4,5-trihydroxy-tetrahydropyran-2-yl]oxy-4-hydroxy-6-(hydroxymethyl)tetrahydropyran-2-yl]oxy-4,5-dihydroxy-6-(hydroxymethyl)tetrahydropyran-2-yl]oxy-3,5-dihydroxy-tetrahydropyran-2-yl]methoxy]-4,5-dihydroxy-6-(hydroxymethyl)tetrahydropyran-3-yl]oxy-4-hydroxy-2-(hydroxymethyl)tetrahydropyran-3-yl]oxy-3,4,5-trihydroxy-tetrahydropyran-2-yl]methoxy]-4-hydroxy-6-[(1R,2R)-1,2,3-trihydroxypropyl]tetrahydropyran-2-carboxylic acid
  REGION 18..19: note = 3-[2-[2-[2-[2-[2-[2-[2-[2-[2-[2-[2-(2-Aminoethoxy)ethoxy]ethoxy]ethoxy]ethoxy]ethoxy]ethoxy]ethoxy]ethoxy]ethoxy]ethoxy]ethoxy]propanoic acid
  SITE 1..12: note = Thiol group of cysteine is linked to N-terminal end of 3-(2-Naphthyl)-L-alanine via -CH2-CO-
  SITE 20: note = Amidation of C-terminal carboxyl group
  SITE 20: note = Lysine side chain is modified with maleimide
XRSGXNWVRWXCGGGGXXXK

SEQ ID NO: 69 - protein, 20 aa, synthetic construct
  REGION 1..20: note = Peptide-69
  SITE 1: note = 3-(2-Naphthyl)-L-alanine
  SITE 5: note = (2S)-2-Amino-4-guanidino-butanoic acid
  SITE 11: note = L-Cyclopentylglycine
  SITE 17: note = 3-[2-[2-[2-[2-[2-[2-[2-[2-[2-[2-[2-(2-Aminoethoxy)ethoxy]ethoxy]ethoxy]ethoxy]ethoxy]ethoxy]ethoxy]ethoxy]ethoxy]ethoxy]ethoxy]propanoic acid
  SITE 18: note = (2R,4S,5R,6R)-5-acetamido-2-[[(2R,3R,4S,5R,6S)-6-[(2R,3S,4R,5R,6S)-5-acetamido-6-[(2S,3S,4S,5S,6R)-2-[[(2R,3R,4S,5S,6S)-6-[(2R,3S,4R,5R,6S)-5-acetamido-6-[(2R,3S,4R,5R,6R)-5-acetamido-6-[2-[[(5S)-5-amino-5-carboxy-pentyl]amino]-2-oxo-ethoxy]-4-hydroxy-2-(hydroxymethyl)tetrahydropyran-3-yl]oxy-4-hydroxy-2-(hydroxymethyl)tetrahydropyran-3-yl]oxy-4-[(2R,3S,4S,5S,6R)-3-[(2S,3R,4R,5S,6R)-3-acetamido-5-[(2S,3R,4S,5R,6R)-6-[[(2R,4S,5R,6R)-5-acetamido-2-carboxy-4-hydroxy-6-[(1R,2R)-1,2,3-trihydroxypropyl]tetrahydropyran-2-yl]oxymethyl]-3,4,5-trihydroxy-tetrahydropyran-2-yl]oxy-4-hydroxy-6-(hydroxymethyl)tetrahydropyran-2-yl]oxy-4,5-dihydroxy-6-(hydroxymethyl)tetrahydropyran-2-yl]oxy-3,5-dihydroxy-tetrahydropyran-2-yl]methoxy]-4,5-dihydroxy-6-(hydroxymethyl)tetrahydropyran-3-yl]oxy-4-hydroxy-2-(hydroxymethyl)tetrahydropyran-3-yl]oxy-3,4,5-trihydroxy-tetrahydropyran-2-yl]methoxy]-4-hydroxy-6-[(1R,2R)-1,2,3-trihydroxypropyl]tetrahydropyran-2-carboxylic acid
  SITE 19: note = 3-[2-[2-[2-[2-[2-[2-[2-[2-[2-[2-[2-(2-Aminoethoxy)ethoxy]ethoxy]ethoxy]ethoxy]ethoxy]ethoxy]ethoxy]ethoxy]ethoxy]ethoxy]ethoxy]propanoic acid
  SITE 1..12: note = Thiol group of cysteine is linked to N-terminal end of 3-(2-Naphthyl)-L-alanine via -CH2-CO-
  SITE 20: note = Amidation of C-terminal carboxyl group
  SITE 20: note = Lysine side chain is modified with maleimide
XRSGXNWVRWXCGGGGXXXK

SEQ ID NO: 70 - protein, 22 aa, synthetic construct
  REGION 1..22: note = Peptide-70
  SITE 1: note = 3-(2-Naphthyl)-L-alanine
  SITE 5: note = (2S)-2-Amino-4-guanidino-butanoic acid
  SITE 8: note = Nle
  SITE 11: note = L-Alpha-cyclohexylglycine
  REGION 13..16: note = MeGly
  SITE 19: note = 3-[2-[2-[2-[2-[2-[2-[2-[2-[2-[2-[2-(2-Aminoethoxy)ethoxy]ethoxy]ethoxy]ethoxy]ethoxy]ethoxy]ethoxy]ethoxy]ethoxy]ethoxy]ethoxy]propanoic acid
  SITE 20: note = (2S)-6-amino-2-[[2-[2-[2-[2-[2-[2-[2-[2-[2-[2-(2-methoxyethoxy)ethoxy]ethoxy]ethoxy]ethoxy]ethoxy]ethoxy]ethoxy]ethoxy]ethoxy]acetyl]amino]hexanoic acid
  SITE 21: note = 3-[2-[2-[2-[2-[2-[2-[2-[2-[2-[2-[2-(2-Aminoethoxy)ethoxy]ethoxy]ethoxy]ethoxy]ethoxy]ethoxy]ethoxy]ethoxy]ethoxy]ethoxy]ethoxy]propanoic acid
  SITE 1..12: note = Thiol group of cysteine is linked to N-terminal end of 3-(2-Naphthyl)-L-alanine via -CH2-CO-
  SITE 22: note = Amidation of C-terminal carboxyl group
  SITE 22: note = Lysine side chain is modified with maleimide
XRSGXNWXRWXCXXXXDDXXXK

SEQ ID NO: 71 - protein, 22 aa, synthetic construct
  REGION 1..22: note = Peptide-71
  SITE 1: note = 3-(2-Naphthyl)-L-alanine
  SITE 5: note = (2S)-2-Amino-4-guanidino-butanoic acid
  SITE 8: note = Nle
  SITE 11: note = L-Alpha-cyclohexylglycine
  SITE 19: note = (2S)-6-amino-2-[[2-[2-[2-[2-[2-[2-[2-[2-[2-[2-(2-methoxyethoxy)ethoxy]ethoxy]ethoxy]ethoxy]ethoxy]ethoxy]ethoxy]ethoxy]ethoxy]acetyl]amino]hexanoic acid
  REGION 20..21: note = 3-[2-[2-[2-[2-[2-[2-[2-[2-[2-[2-[2-(2-Aminoethoxy)ethoxy]ethoxy]ethoxy]ethoxy]ethoxy]ethoxy]ethoxy]ethoxy]ethoxy]ethoxy]ethoxy]propanoic acid
  SITE 1..12: note = Thiol group of cysteine is linked to N-terminal end of 3-(2-Naphthyl)-L-alanine via -CH2-CO-
  SITE 22: note = Amidation of C-terminal carboxyl group
  SITE 22: note = Lysine side chain is modified with maleimide
XRSGXNWXRWXCGSGSDDXXXK

SEQ ID NO: 72 - protein, 22 aa, synthetic construct
  REGION 1..22: note = Peptide-72
  SITE 1: note = 3-(2-Naphthyl)-L-alanine
  SITE 5: note = (2S)-2-Amino-4-guanidino-butanoic acid
  SITE 8: note = Nle
  SITE 11: note = L-Alpha-cyclohexylglycine
  SITE 19: note = 3-[2-[2-[2-[2-[2-[2-[2-[2-[2-[2-[2-(2-Aminoethoxy)ethoxy]ethoxy]ethoxy]ethoxy]ethoxy]ethoxy]ethoxy]ethoxy]ethoxy]ethoxy]ethoxy]propanoic acid
  SITE 20: note = (2S)-6-amino-2-[[2-[2-[2-[2-[2-[2-[2-[2-[2-[2-(2-methoxyethoxy)ethoxy]ethoxy]ethoxy]ethoxy]ethoxy]ethoxy]ethoxy]ethoxy]ethoxy]acetyl]amino]hexanoic acid
  SITE 21: note = 3-[2-[2-[2-[2-[2-[2-[2-[2-[2-[2-[2-(2-Aminoethoxy)ethoxy]ethoxy]ethoxy]ethoxy]ethoxy]ethoxy]ethoxy]ethoxy]ethoxy]ethoxy]ethoxy]propanoic acid
  SITE 1..12: note = Thiol group of cysteine is linked to N-terminal end of 3-(2-Naphthyl)-L-alanine via -CH2-CO-
  SITE 22: note = Amidation of C-terminal carboxyl group
  SITE 22: note = Lysine side chain is modified with maleimide
XRSGXNWXRWXCGSGSDDXXXK

SEQ ID NO: 73 - protein, 18 aa, synthetic construct
  REGION 1..18: note = Peptide-73
  SITE 1: note = 3-(2-Naphthyl)-L-alanine
  SITE 17: note = 3-[2-[2-[2-[2-[2-[2-[2-[2-[2-[2-[2-(2-Aminoethoxy)ethoxy]ethoxy]ethoxy]ethoxy]ethoxy]ethoxy]ethoxy]ethoxy]ethoxy]ethoxy]ethoxy]propanoic acid
  SITE 1..12: note = Thiol group of cysteine is linked to N-terminal end of 3-(2-Naphthyl)-L-alanine via -CH2-CO-
  SITE 18: note = Amidation of C-terminal carboxyl group
  SITE 18: note = Lysine side chain is modified with DBCO
XRSGRNWVVWVCGGGGXK

SEQ ID NO: 74 - protein, 18 aa, synthetic construct
  REGION 1..18: note = Peptide-74
  SITE 1: note = 3-(2-Naphthyl)-L-alanine
  SITE 5: note = (2S)-2-Amino-4-guanidino-butanoic acid
  SITE 11: note = L-Cyclopentylglycine
  SITE 17: note = 3-[2-[2-[2-[2-[2-[2-[2-[2-[2-[2-[2-(2-Aminoethoxy)ethoxy]ethoxy]ethoxy]ethoxy]ethoxy]ethoxy]ethoxy]ethoxy]ethoxy]ethoxy]ethoxy]propanoic acid
  SITE 1..12: note = Thiol group of cysteine is linked to N-terminal end of 3-(2-Naphthyl)-L-alanine via -CH2-CO-
  SITE 18: note = Amidation of C-terminal carboxyl group
  SITE 18: note = Lysine side chain is modified with DBCO
XRSGXNWVRWXCGGGGXK

SEQ ID NO: 75 - protein, 20 aa, synthetic construct
  REGION 1..20: note = Peptide-75
  SITE 1: note = 3-(2-Naphthyl)-L-alanine
  SITE 5: note = (2S)-2-Amino-4-guanidino-butanoic acid
  SITE 11: note = L-Cyclopentylglycine
  SITE 19: note = 3-[2-[2-[2-[2-[2-[2-[2-[2-[2-[2-[2-(2-Aminoethoxy)ethoxy]ethoxy]ethoxy]ethoxy]ethoxy]ethoxy]ethoxy]ethoxy]ethoxy]ethoxy]ethoxy]propanoic acid
  SITE 1..12: note = Thiol group of cysteine is linked to N-terminal end of 3-(2-Naphthyl)-L-alanine via -CH2-CO-
  SITE 20: note = Amidation of C-terminal carboxyl group
  SITE 20: note = Lysine side chain is modified with DBCO
XRSGXNWVRWXCGGGGDDXK

SEQ ID NO: 76 - protein, 20 aa, synthetic construct
  REGION 1..20: note = Peptide-76
  SITE 1: note = 3-(2-Naphthyl)-L-alanine
  SITE 3: note = L-Homocysteine
  SITE 8: note = L-Homocysteine
  SITE 11: note = L-Cyclopentylglycine
  SITE 19: note = 3-[2-[2-[2-[2-[2-[2-[2-[2-[2-[2-[2-(2-Aminoethoxy)ethoxy]ethoxy]ethoxy]ethoxy]ethoxy]ethoxy]ethoxy]ethoxy]ethoxy]ethoxy]ethoxy]propanoic acid
  SITE 1..12: note = Thiol group of cysteine is linked to N-terminal end of 3-(2-Naphthyl)-L-alanine via -CH2-CO-
  SITE 3..8: note = Thiol groups are linked as a disulfide
  SITE 20: note = Amidation of C-terminal carboxyl group
  SITE 20: note = Lysine side chain is modified with DBCO
XRXGRDWXRWXCGGGGDDXK

SEQ ID NO: 77 - protein, 21 aa, synthetic construct
  REGION 1..21: note = Peptide-77
  SITE 1: note = 3-(2-Naphthyl)-L-alanine
  SITE 3: note = L-Homocysteine
  SITE 5: note = (2S)-2-Amino-4-guanidino-butanoic acid
  SITE 8: note = L-Homocysteine
  SITE 11: note = L-Cyclopentylglycine
  SITE 20: note = 3-[2-[2-[2-[2-[2-[2-[2-[2-[2-[2-[2-(2-Aminoethoxy)ethoxy]ethoxy]ethoxy]ethoxy]ethoxy]ethoxy]ethoxy]ethoxy]ethoxy]ethoxy]ethoxy]propanoic acid
  SITE 1..12: note = Thiol group of cysteine is linked to N-terminal end of 3-(2-Naphthyl)-L-alanine via -CH2-CO-
  SITE 3..8: note = Thiol groups are linked as a disulfide
  SITE 21: note = Amidation of C-terminal carboxyl group
  SITE 21: note = Lysine side chain is modified with DBCO
XRXGXNWXRWXCGGGGDDDXK

SEQ ID NO: 78 - protein, 20 aa, synthetic construct
  REGION 1..20: note = Peptide-78
  SITE 1: note = 3-(2-Naphthyl)-L-alanine
  SITE 3: note = L-Homocysteine
  SITE 5: note = (2S)-2-Amino-4-guanidino-butanoic acid
  SITE 8: note = L-Homocysteine
  SITE 11: note = L-Cyclopentylglycine
  SITE 19: note = 3-[2-[2-[2-[2-[2-[2-[2-[2-[2-[2-[2-(2-Aminoethoxy)ethoxy]ethoxy]ethoxy]ethoxy]ethoxy]ethoxy]ethoxy]ethoxy]ethoxy]ethoxy]ethoxy]propanoic acid
  SITE 1..12: note = Thiol group of cysteine is linked to N-terminal end of 3-(2-Naphthyl)-L-alanine via -CH2-CO-
  SITE 3..8: note = Thiol groups are linked as a disulfide
  SITE 20: note = Amidation of C-terminal carboxyl group
  SITE 20: note = Lysine side chain is modified with DBCO
XRXGXDWXRWXCGGGGDDXK

SEQ ID NO: 79 - protein, 20 aa, synthetic construct
  REGION 1..20: note = Peptide-79
  SITE 1: note = 3-(2-Naphthyl)-L-alanine
  SITE 5: note = (2S)-2-Amino-4-guanidino-butanoic acid
  SITE 8: note = Nle
  SITE 11: note = L-Alpha-cyclohexylglycine
  SITE 19: note = 3-[2-[2-[2-[2-[2-[2-[2-[2-[2-[2-[2-(2-Aminoethoxy)ethoxy]ethoxy]ethoxy]ethoxy]ethoxy]ethoxy]ethoxy]ethoxy]ethoxy]ethoxy]ethoxy]propanoic acid
  SITE 1..12: note = Thiol group of cysteine is linked to N-terminal end of 3-(2-Naphthyl)-L-alanine via -CH2-CO-
  SITE 20: note = Amidation of C-terminal carboxyl group
  SITE 20: note = Lysine side chain is modified with DBCO
XRSGXNWXRWXCGGGGDDXK

SEQ ID NO: 80 - protein, 21 aa, synthetic construct
  REGION 1..21: note = Peptide-80
  SITE 1: note = 3-(2-Naphthyl)-L-alanine
  SITE 20: note = 3-[2-[2-[2-[2-[2-[2-[2-[2-[2-[2-[2-(2-Aminoethoxy)ethoxy]ethoxy]ethoxy]ethoxy]ethoxy]ethoxy]ethoxy]ethoxy]ethoxy]ethoxy]ethoxy]propanoic acid
  SITE 1..12: note = Thiol group of cysteine is linked to N-terminal end of 3-(2-Naphthyl)-L-alanine via -CH2-CO-
  SITE 21: note = Amidation of C-terminal carboxyl group
  SITE 21: note = Lysine side chain is modified with DBCO
XRSGRNWVVWVCGGGGDDDXK

SEQ ID NO: 81 - protein, 18 aa, synthetic construct
  REGION 1..18: note = Peptide-81
  SITE 1: note = 3-(2-Naphthyl)-L-alanine
  SITE 11: note = L-Cyclopentylglycine
  SITE 17: note = 3-[2-[2-[2-[2-[2-[2-[2-[2-[2-[2-[2-(2-Aminoethoxy)ethoxy]ethoxy]ethoxy]ethoxy]ethoxy]ethoxy]ethoxy]ethoxy]ethoxy]ethoxy]ethoxy]propanoic acid
  SITE 1..12: note = Thiol group of cysteine is linked to N-terminal end of 3-(2-Naphthyl)-L-alanine via -CH2-CO-
  SITE 18: note = Amidation of C-terminal carboxyl group
  SITE 18: note = Lysine side chain is modified with DBCO
XRSGRNWVRWXCGGGGXK

SEQ ID NO: 82 - protein, 30 aa, synthetic construct
  REGION 1..18: note = Peptide-82
  SITE 1: note = 3-(2-Naphthyl)-L-alanine
  SITE 17..29: note = MeGly
  SITE 1..12: note = Thiol group of cysteine is linked to N-terminal end of 3-(2-Naphthyl)-L-alanine via -CH2-CO-
  SITE 30: note = Amidation of C-terminal carboxyl group
  SITE 30: note = Lysine side chain is modified with DBCO
XRSGRNWVVWVCGGGGXXXXXXXXXXXXXK

SEQ ID NO: 83 - protein, 18 aa, synthetic construct
  REGION 1..18: note = Peptide-83
  SITE 1: note = 3-(2-Naphthyl)-L-alanine
  SITE 9: note = (2S)-2-Amino-4-guanidino-butanoic acid
  SITE 11: note = L-Cyclopentylglycine
  SITE 17: note = 3-[2-[2-[2-[2-[2-[2-[2-[2-[2-[2-[2-(2-Aminoethoxy)ethoxy]ethoxy]ethoxy]ethoxy]ethoxy]ethoxy]ethoxy]ethoxy]ethoxy]ethoxy]ethoxy]propanoic acid
  SITE 1..12: note = Thiol group of cysteine is linked to N-terminal end of 3-(2-Naphthyl)-L-alanine via -CH2-CO-
  SITE 18: note = Amidation of C-terminal carboxyl group
  SITE 18: note = Lysine side chain is modified with DBCO
XRSGRDWVXWXCGGGGXK

SEQ ID NO: 84 - protein, 18 aa, synthetic construct
  REGION 1..18: note = Peptide-84
  SITE 1: note = 3-(2-Naphthyl)-L-alanine
  SITE 3: note = L-Homocysteine
  SITE 8: note = L-Homocysteine
  SITE 17: note = 3-[2-[2-[2-[2-[2-[2-[2-[2-[2-[2-[2-(2-Aminoethoxy)ethoxy]ethoxy]ethoxy]ethoxy]ethoxy]ethoxy]ethoxy]ethoxy]ethoxy]ethoxy]ethoxy]propanoic acid
  SITE 1..12: note = Thiol group of cysteine is linked to N-terminal end of 3-(2-Naphthyl)-L-alanine via -CH2-CO-
  SITE 3..8: note = Thiol groups are linked as a disulfide
  SITE 18: note = Amidation of C-terminal carboxyl group
  SITE 18: note = Lysine side chain is modified with DBCO
XRXGRNWXVWVCGGGGXK

SEQ ID NO: 85 - protein, 18 aa, synthetic construct
  REGION 1..18: note = Peptide-85
  SITE 1: note = 3-(2-Naphthyl)-L-alanine
  SITE 8: note = Nle
  SITE 11: note = L-Cyclopentylglycine
  SITE 17: note = 3-[2-[2-[2-[2-[2-[2-[2-[2-[2-[2-[2-(2-Aminoethoxy)ethoxy]ethoxy]ethoxy]ethoxy]ethoxy]ethoxy]ethoxy]ethoxy]ethoxy]ethoxy]ethoxy]propanoic acid
  SITE 1..12: note = Thiol group of cysteine is linked to N-terminal end of 3-(2-Naphthyl)-L-alanine via -CH2-CO-
  SITE 18: note = Amidation of C-terminal carboxyl group
  SITE 18: note = Lysine side chain is modified with DBCO
XRSGRNWXVWXCGGGGXK

SEQ ID NO: 86 - protein, 18 aa, synthetic construct
  REGION 1..18: note = Peptide-86
  SITE 1: note = 3-(2-Naphthyl)-L-alanine
  SITE 3: note = L-Homocysteine
  SITE 5: note = (2S)-2-Amino-4-guanidino-butanoic acid
  SITE 8: note = L-Homocysteine
  SITE 11: note = L-Cyclopentylglycine
  SITE 17: note = 3-[2-[2-[2-[2-[2-[2-[2-[2-[2-[2-[2-(2-Aminoethoxy)ethoxy]ethoxy]ethoxy]ethoxy]ethoxy]ethoxy]ethoxy]ethoxy]ethoxy]ethoxy]ethoxy]propanoic acid
  SITE 1..12: note = Thiol group of cysteine is linked to N-terminal end of 3-(2-Naphthyl)-L-alanine via -CH2-CO-
  SITE 3..8: note = Thiol groups are linked as a disulfide
  SITE 18: note = Amidation of C-terminal carboxyl group
  SITE 18: note = Lysine side chain is modified with DBCO
XRXGXNWXRWXCGGGGXK

SEQ ID NO: 87 - protein, 18 aa, synthetic construct
  REGION 1..18: note = Peptide-87
  SITE 1: note = 3-(2-Naphthyl)-L-alanine
  SITE 2: note = L-Tert-Leucine
  SITE 11: note = L-Cyclopentylglycine
  SITE 17: note = 3-[2-[2-[2-[2-[2-[2-[2-[2-[2-[2-[2-(2-Aminoethoxy)ethoxy]ethoxy]ethoxy]ethoxy]ethoxy]ethoxy]ethoxy]ethoxy]ethoxy]ethoxy]ethoxy]propanoic acid
  SITE 1..12: note = Thiol group of cysteine is linked to N-terminal end of 3-(2-Naphthyl)-L-alanine via -CH2-CO-
  SITE 18: note = Amidation of C-terminal carboxyl group
  SITE 18: note = Lysine side chain is modified with DBCO
XXSGRNWVRWXCGGGGXK

SEQ ID NO: 88 - protein, 22 aa, synthetic construct
  REGION 1..22: note = Peptide-88
  SITE 1: note = 3-(2-Naphthyl)-L-alanine
  SITE 5: note = (2S)-2-Amino-4-guanidino-butanoic acid
  SITE 11: note = L-Cyclopentylglycine
  SITE 21: note = 3-[2-[2-[2-[2-[2-[2-[2-[2-[2-[2-[2-(2-Aminoethoxy)ethoxy]ethoxy]ethoxy]ethoxy]ethoxy]ethoxy]ethoxy]ethoxy]ethoxy]ethoxy]ethoxy]propanoic acid
  SITE 1..12: note = Thiol group of cysteine is linked to N-terminal end of 3-(2-Naphthyl)-L-alanine via -CH2-CO-
  SITE 22: note = Amidation of C-terminal carboxyl group
  SITE 22: note = Lysine side chain is modified with DBCO
XRSGXNWVRWXCGGGGDDDDXK

SEQ ID NO: 89 - protein, 21 aa, synthetic construct
  REGION 1..21: note = Peptide-89
  SITE 1: note = 3-(2-Naphthyl)-L-alanine
  SITE 5: note = (2S)-2-Amino-4-guanidino-butanoic acid
  SITE 11: note = L-Cyclopentylglycine
  SITE 20: note = 3-[2-[2-[2-[2-[2-[2-[2-[2-[2-[2-[2-(2-Aminoethoxy)ethoxy]ethoxy]ethoxy]ethoxy]ethoxy]ethoxy]ethoxy]ethoxy]ethoxy]ethoxy]ethoxy]propanoic acid
  SITE 1..12: note = Thiol group of cysteine is linked to N-terminal end of 3-(2-Naphthyl)-L-alanine via -CH2-CO-
  SITE 21: note = Amidation of C-terminal carboxyl group
  SITE 21: note = Lysine side chain is modified with DBCO
XRSGXNWVRWXCGGGGDDDXK

SEQ ID NO: 90 - protein, 20 aa, synthetic construct
  REGION 1..20: note = Peptide-90
  SITE 1: note = 3-(2-Naphthyl)-L-alanine
  SITE 5: note = (2S)-2-Amino-4-guanidino-butanoic acid
  SITE 11: note = L-Cyclopentylglycine
  SITE 18: note = 3-[2-[2-[2-[2-[2-[2-[2-[2-[2-[2-[2-(2-Aminoethoxy)ethoxy]ethoxy]ethoxy]ethoxy]ethoxy]ethoxy]ethoxy]ethoxy]ethoxy]ethoxy]ethoxy]propanoic acid
  SITE 1..12: note = Thiol group of cysteine is linked to N-terminal end of 3-(2-Naphthyl)-L-alanine via -CH2-CO-
  SITE 20: note = Amidation of C-terminal carboxyl group
  SITE 20: note = Lysine side chain is modified with DBCO
XRSGXNWVRWXCGGGGDXDK

SEQ ID NO: 91 - protein, 20 aa, synthetic construct
  REGION 1..20: note = Peptide-91
  SITE 1: note = 3-(2-Naphthyl)-L-alanine
  SITE 5: note = (2S)-2-Amino-4-guanidino-butanoic acid
  SITE 11: note = L-Alpha-cyclohexylglycine
  SITE 19: note = 3-[2-[2-[2-[2-[2-[2-[2-[2-[2-[2-[2-(2-Aminoethoxy)ethoxy]ethoxy]ethoxy]ethoxy]ethoxy]ethoxy]ethoxy]ethoxy]ethoxy]ethoxy]ethoxy]propanoic acid
  SITE 1..12: note = Thiol group of cysteine is linked to N-terminal end of 3-(2-Naphthyl)-L-alanine via -CH2-CO-
  SITE 20: note = Amidation of C-terminal carboxyl group
  SITE 20: note = Lysine side chain is modified with DBCO
XRSGXNWVRWXCGGGGDDXK

SEQ ID NO: 92 - protein, 20 aa, synthetic construct
  REGION 1..20: note = Peptide-92
  SITE 1: note = 3-(2-Naphthyl)-L-alanine
  SITE 3: note = L-Homocysteine
  SITE 5: note = (2S)-2-Amino-4-guanidino-butanoic acid
  SITE 8: note = L-Homocysteine
  SITE 11: note = L-Cyclopentylglycine
  SITE 19: note = 3-[2-[2-[2-[2-[2-[2-[2-[2-[2-[2-[2-(2-Aminoethoxy)ethoxy]ethoxy]ethoxy]ethoxy]ethoxy]ethoxy]ethoxy]ethoxy]ethoxy]ethoxy]ethoxy]propanoic acid
  SITE 1..12: note = Thiol group of cysteine is linked to N-terminal end of 3-(2-Naphthyl)-L-alanine via -CH2-CO-
  SITE 3..8: note = Thiol groups are linked as a disulfide
  SITE 20: note = Amidation of C-terminal carboxyl group
  SITE 20: note = Lysine side chain is modified with DBCO
XRXGXNWXRWXCGGGGDDXK

SEQ ID NO: 93 - protein, 19 aa, synthetic construct
  REGION 1..19: note = Peptide-93
  SITE 1: note = 3-(2-Naphthyl)-L-alanine
  SITE 3: note = L-Homocysteine
  SITE 5: note = (2S)-2-Amino-4-guanidino-butanoic acid
  SITE 8: note = L-Homocysteine
  SITE 11: note = L-Cyclopentylglycine
  SITE 18: note = 3-[2-[2-[2-[2-[2-[2-[2-[2-[2-[2-[2-(2-Aminoethoxy)ethoxy]ethoxy]ethoxy]ethoxy]ethoxy]ethoxy]ethoxy]ethoxy]ethoxy]ethoxy]ethoxy]propanoic acid
  SITE 1..12: note = Thiol group of cysteine is linked to N-terminal end of 3-(2-Naphthyl)-L-alanine via -CH2-CO-
  SITE 3..8: note = Thiol groups are linked as a disulfide
  SITE 19: note = Amidation of C-terminal carboxyl group
  SITE 19: note = Lysine side chain is modified with DBCO
XRXGXNWXRWXCGGGGDXK

SEQ ID NO: 94 - protein, 20 aa, synthetic construct
  REGION 1..20: note = Peptide-94
  SITE 1: note = 3-(2-Naphthyl)-L-alanine
  SITE 3: note = L-Homocysteine
  SITE 5: note = (2S)-2-Amino-4-guanidino-butanoic acid
  SITE 8: note = L-Homocysteine
  SITE 11: note = L-Cyclopentylglycine
  SITE 18: note = 3-[2-[2-[2-[2-[2-[2-[2-[2-[2-[2-[2-(2-Aminoethoxy)ethoxy]ethoxy]ethoxy]ethoxy]ethoxy]ethoxy]ethoxy]ethoxy]ethoxy]ethoxy]ethoxy]propanoic acid
  SITE 1..12: note = Thiol group of cysteine is linked to N-terminal end of 3-(2-Naphthyl)-L-alanine via -CH2-CO-
  SITE 3..8: note = Thiol groups are linked as a disulfide
  SITE 20: note = Amidation of C-terminal carboxyl group
  SITE 20: note = Lysine side chain is modified with DBCO
XRXGXNWXRWXCGGGGDXDK

SEQ ID NO: 95 - protein, 20 aa, synthetic construct
  REGION 1..20: note = Peptide-95
  SITE 1: note = 3-(2-Naphthyl)-L-alanine
  SITE 11: note = L-Cyclopentylglycine
  SITE 19: note = 3-[2-[2-[2-[2-[2-[2-[2-[2-[2-[2-[2-(2-Aminoethoxy)ethoxy]ethoxy]ethoxy]ethoxy]ethoxy]ethoxy]ethoxy]ethoxy]ethoxy]ethoxy]ethoxy]propanoic acid
  SITE 1..12: note = Thiol group of cysteine is linked to N-terminal end of 3-(2-Naphthyl)-L-alanine via -CH2-CO-
  SITE 20: note = Amidation of C-terminal carboxyl group
  SITE 20: note = Lysine side chain is modified with DBCO
XRSGRNWVRWXCGGGGDDXK

SEQ ID NO: 96 - protein, 19 aa, synthetic construct
  REGION 1..19: note = Peptide-96
  SITE 1: note = 3-(2-Naphthyl)-L-alanine
  SITE 11: note = L-Cyclopentylglycine
  SITE 18: note = 3-[2-[2-[2-[2-[2-[2-[2-[2-[2-[2-[2-(2-Aminoethoxy)ethoxy]ethoxy]ethoxy]ethoxy]ethoxy]ethoxy]ethoxy]ethoxy]ethoxy]ethoxy]ethoxy]propanoic acid
  SITE 1..12: note = Thiol group of cysteine is linked to N-terminal end of 3-(2-Naphthyl)-L-alanine via -CH2-CO-
  SITE 19: note = Amidation of C-terminal carboxyl group
  SITE 19: note = Lysine side chain is modified with DBCO
XRSGRDWVRWXCGGGGDXK

SEQ ID NO: 97 - protein, 19 aa, synthetic construct
  REGION 1..19: note = Peptide-97
  SITE 1: note = 3-(2-Naphthyl)-L-alanine
  SITE 11: note = L-Cyclopentylglycine
  SITE 18: note = 3-[2-[2-[2-[2-[2-[2-[2-[2-[2-[2-[2-(2-Aminoethoxy)ethoxy]ethoxy]ethoxy]ethoxy]ethoxy]ethoxy]ethoxy]ethoxy]ethoxy]ethoxy]ethoxy]propanoic acid
  SITE 1..12: note = Thiol group of cysteine is linked to N-terminal end of 3-(2-Naphthyl)-L-alanine via -CH2-CO-
  SITE 19: note = Lysine side chain is modified with DBCO
XRSGRNWVRWXCGGGGDXK

SEQ ID NO: 98 - protein, 20 aa, synthetic construct
  REGION 1..20: note = Peptide-98
  SITE 1: note = 3-(2-Naphthyl)-L-alanine
  SITE 11: note = L-Cyclopentylglycine
  SITE 19: note = 3-[2-[2-[2-[2-[2-[2-[2-[2-[2-[2-[2-(2-Aminoethoxy)ethoxy]ethoxy]ethoxy]ethoxy]ethoxy]ethoxy]ethoxy]ethoxy]ethoxy]ethoxy]ethoxy]propanoic acid
  SITE 1..12: note = Thiol group of cysteine is linked to N-terminal end of 3-(2-Naphthyl)-L-alanine via -CH2-CO-
  SITE 20: note = Amidation of C-terminal carboxyl group
  SITE 20: note = Lysine side chain is modified with DBCO
XRSGRNWVRWXCGGEGGEXK

SEQ ID NO: 99 - protein, 20 aa, synthetic construct
  REGION 1..20: note = Peptide-99
  SITE 1: note = 3-(2-Naphthyl)-L-alanine
  SITE 3: note = L-Homocysteine
  SITE 8: note = L-Homocysteine
  SITE 11: note = L-Cyclopentylglycine
  SITE 19: note = 3-[2-[2-[2-[2-[2-[2-[2-[2-[2-[2-[2-(2-Aminoethoxy)ethoxy]ethoxy]ethoxy]ethoxy]ethoxy]ethoxy]ethoxy]ethoxy]ethoxy]ethoxy]ethoxy]propanoic acid
  SITE 1..12: note = Thiol group of cysteine is linked to N-terminal end of 3-(2-Naphthyl)-L-alanine via -CH2-CO-
  SITE 3..8: note = Thiol groups are linked as a disulfide
  SITE 20: note = Lysine side chain is modified with DBCO
XRXGRNWXRWXCGGGGDDXK

SEQ ID NO: 100 - protein, 20 aa, synthetic construct
  REGION 1..20: note = Peptide-100
  SITE 1: note = 3-(2-Naphthyl)-L-alanine
  SITE 5: note = (2S)-2-Amino-4-guanidino-butanoic acid
  SITE 11: note = L-Cyclopentylglycine
  SITE 17: note = 3-[2-[2-[2-[2-[2-[2-[2-[2-[2-[2-[2-(2-Aminoethoxy)ethoxy]ethoxy]ethoxy]ethoxy]ethoxy]ethoxy]ethoxy]ethoxy]ethoxy]ethoxy]ethoxy]propanoic acid
  SITE 1..12: note = Thiol group of cysteine is linked to N-terminal end of 3-(2-Naphthyl)-L-alanine via -CH2-CO-
  SITE 20: note = Amidation of C-terminal carboxyl group
  SITE 20: note = Lysine side chain is modified with DBCO
XRSGXNWVRWXCGGGGXDDK

SEQ ID NO: 101 - protein, 20 aa, synthetic construct
  REGION 1..20: note = Peptide-101
  SITE 1: note = 3-(2-Naphthyl)-L-alanine
  SITE 5: note = (2S)-2-Amino-4-guanidino-butanoic acid
  SITE 11: note = L-Cyclopentylglycine
  REGION 13..16: note = bAla
  SITE 19: note = 3-[2-[2-[2-[2-[2-[2-[2-[2-[2-[2-[2-(2-Aminoethoxy)ethoxy]ethoxy]ethoxy]ethoxy]ethoxy]ethoxy]ethoxy]ethoxy]ethoxy]ethoxy]ethoxy]propanoic acid
  SITE 1..12: note = Thiol group of cysteine is linked to N-terminal end of 3-(2-Naphthyl)-L-alanine via -CH2-CO-
  SITE 20: note = Amidation of C-terminal carboxyl group
  SITE 20: note = Lysine side chain is modified with DBCO
XRSGXNWVRWXCXXXXDDXK

SEQ ID NO: 102 - protein, 20 aa, synthetic construct
  REGION 1..20: note = Peptide-102
  SITE 1: note = 3-(2-Naphthyl)-L-alanine
  SITE 5: note = (2S)-2-Amino-4-guanidino-butanoic acid
  SITE 11: note = L-Cyclopentylglycine
  REGION 17..18: note = D-Aspartic acid
  SITE 19: note = 3-[2-[2-[2-[2-[2-[2-[2-[2-[2-[2-[2-(2-Aminoethoxy)ethoxy]ethoxy]ethoxy]ethoxy]ethoxy]ethoxy]ethoxy]ethoxy]ethoxy]ethoxy]ethoxy]propanoic acid
  SITE 1..12: note = Thiol group of cysteine is linked to N-terminal end of 3-(2-Naphthyl)-L-alanine via -CH2-CO-
  SITE 20: note = Amidation of C-terminal carboxyl group
  SITE 20: note = Lysine side chain is modified with DBCO
XRSGXNWVRWXCGGGGXXXK

SEQ ID NO: 103 - protein, 20 aa, synthetic construct
  REGION 1..20: note = Peptide-103
  SITE 1: note = 3-(2-Naphthyl)-L-alanine
  SITE 5: note = (2S)-2-Amino-4-guanidino-butanoic acid
  SITE 11: note = L-Cyclopentylglycine
  REGION 13..16: note = bAla
  REGION 17..18: note = D-Aspartic acid
  SITE 19: note = 3-[2-[2-[2-[2-[2-[2-[2-[2-[2-[2-[2-(2-Aminoethoxy)ethoxy]ethoxy]ethoxy]ethoxy]ethoxy]ethoxy]ethoxy]ethoxy]ethoxy]ethoxy]ethoxy]propanoic acid
  SITE 1..12: note = Thiol group of cysteine is linked to N-terminal end of 3-(2-Naphthyl)-L-alanine via -CH2-CO-
  SITE 20: note = Amidation of C-terminal carboxyl group
  SITE 20: note = Lysine side chain is modified with DBCO
XRSGXNWVRWXCXXXXXXXK

SEQ ID NO: 104 - protein, 18 aa, synthetic construct
  REGION 1..18: note = Peptide-104
  SITE 1: note = 3-(2-Naphthyl)-L-alanine
  SITE 8: note = Nle
  SITE 11: note = L-Alpha-cyclohexylglycine
  SITE 17: note = 3-[2-[2-[2-[2-[2-[2-[2-[2-[2-[2-[2-(2-Aminoethoxy)ethoxy]ethoxy]ethoxy]ethoxy]ethoxy]ethoxy]ethoxy]ethoxy]ethoxy]ethoxy]ethoxy]propanoic acid
  SITE 1..12: note = Thiol group of cysteine is linked to N-terminal end of 3-(2-Naphthyl)-L-alanine via -CH2-CO-
  SITE 18: note = Amidation of C-terminal carboxyl group
  SITE 18: note = Lysine side chain is modified with DBCO
XRSGRNWXVWXCGGGGXK

SEQ ID NO: 105 - protein, 20 aa, synthetic construct
  REGION 1..20: note = Peptide-105
  SITE 1: note = 3-(2-Naphthyl)-L-alanine
  SITE 8: note = Nle
  SITE 11: note = L-Alpha-cyclohexylglycine
  SITE 19: note = 3-[2-[2-[2-[2-[2-[2-[2-[2-[2-[2-[2-(2-Aminoethoxy)ethoxy]ethoxy]ethoxy]ethoxy]ethoxy]ethoxy]ethoxy]ethoxy]ethoxy]ethoxy]ethoxy]propanoic acid
  SITE 1..12: note = Thiol group of cysteine is linked to N-terminal end of 3-(2-Naphthyl)-L-alanine via -CH2-CO-
  SITE 20: note = Amidation of C-terminal carboxyl group
  SITE 20: note = Lysine side chain is modified with DBCO
XRSGRNWXVWXCGGGGDDXK

SEQ ID NO: 106 - protein, 19 aa, synthetic construct
  REGION 1..19: note = Peptide-106
  SITE 1: note = 3-(2-Naphthyl)-L-alanine
  SITE 5: note = (2S)-2-Amino-4-guanidino-butanoic acid
  SITE 11: note = L-Cyclopentylglycine
  SITE 18: note = 3-[2-[2-[2-[2-[2-[2-[2-[2-[2-[2-[2-(2-Aminoethoxy)ethoxy]ethoxy]ethoxy]ethoxy]ethoxy]ethoxy]ethoxy]ethoxy]ethoxy]ethoxy]ethoxy]propanoic acid
  SITE 1..12: note = Thiol group of cysteine is linked to N-terminal end of 3-(2-Naphthyl)-L-alanine via -CH2-CO-
  SITE 19: note = Amidation of C-terminal carboxyl group
  SITE 19: note = Lysine side chain is modified with DBCO
XRSGXDWVRWXCGGGGDXK

SEQ ID NO: 107 - protein, 18 aa, synthetic construct
  REGION 1..18: note = Peptide-107
  SITE 1: note = 3-(2-Naphthyl)-L-alanine
  SITE 5: note = (2S)-2-Amino-4-guanidino-butanoic acid
  SITE 11: note = L-Cyclopentylglycine
  SITE 17: note = 3-[2-[2-[2-[2-[2-[2-[2-[2-[2-[2-[2-(2-Aminoethoxy)ethoxy]ethoxy]ethoxy]ethoxy]ethoxy]ethoxy]ethoxy]ethoxy]ethoxy]ethoxy]ethoxy]propanoic acid
  SITE 1..12: note = Thiol group of cysteine is linked to N-terminal end of 3-(2-Naphthyl)-L-alanine via -CH2-CO-
  SITE 18: note = Lysine side chain is modified with DBCO
XRSGXDWVRWXCGGGGXK

SEQ ID NO: 108 - protein, 19 aa, synthetic construct
  REGION 1..19: note = Peptide-108
  SITE 1: note = 3-(2-Naphthyl)-L-alanine
  SITE 3: note = L-Homocysteine
  SITE 5: note = (2S)-2-Amino-4-guanidino-butanoic acid
  SITE 8: note = L-Homocysteine
  SITE 11: note = L-Cyclopentylglycine
  SITE 18: note = 3-[2-[2-[2-[2-[2-[2-[2-[2-[2-[2-[2-(2-Aminoethoxy)ethoxy]ethoxy]ethoxy]ethoxy]ethoxy]ethoxy]ethoxy]ethoxy]ethoxy]ethoxy]ethoxy]propanoic acid
  SITE 1..12: note = Thiol group of cysteine is linked to N-terminal end of 3-(2-Naphthyl)-L-alanine via -CH2-CO-
  SITE 3..8: note = Thiol groups are linked as a disulfide
  SITE 19: note = Lysine side chain is modified with DBCO
XRXGXDWXRWXCGGGGDXK

SEQ ID NO: 109 - protein, 20 aa, synthetic construct
  REGION 1..20: note = Peptide-109
  SITE 1: note = 3-(2-Naphthyl)-L-alanine
  SITE 5: note = (2S)-2-Amino-4-guanidino-butanoic acid
  SITE 8: note = Nle
  SITE 11: note = L-Cyclopentylglycine
  SITE 19: note = 3-[2-[2-[2-[2-[2-[2-[2-[2-[2-[2-[2-(2-Aminoethoxy)ethoxy]ethoxy]ethoxy]ethoxy]ethoxy]ethoxy]ethoxy]ethoxy]ethoxy]ethoxy]ethoxy]propanoic acid
  SITE 1..12: note = Thiol group of cysteine is linked to N-terminal end of 3-(2-Naphthyl)-L-alanine via -CH2-CO-
  SITE 20: note = Amidation of C-terminal carboxyl group
  SITE 20: note = Lysine side chain is modified with DBCO
XRSGXNWXRWXCGGGGDDXK

SEQ ID NO: 110 - protein, 12 aa, synthetic construct
  REGION 1..12: note = Peptide-110
  SITE 1: note = 3-(2-Naphthyl)-L-alanine
  SITE 12: note = C-terminal carboxyl group is linked to N-terminal amino group of linker via amide bond
  SITE 1..12: note = Thiol group of cysteine is linked to N-terminal end of 3-(2-Naphthyl)-L-alanine via -CH2-CO-
XRSGRNWVVWVC

SEQ ID NO: 111 - protein, 12 aa, synthetic construct
  REGION 1..12: note = Peptide-111
  SITE 1: note = 3-(2-Naphthyl)-L-alanine
  SITE 12: note = C-terminal carboxyl group is linked to N-terminal amino group of linker via amide bond
  SITE 1..12: note = Thiol group of cysteine is linked to N-terminal end of 3-(2-Naphthyl)-L-alanine via -CH2-CO-
XRSGRNWVRWVC

SEQ ID NO: 112 - protein, 12 aa, synthetic construct
  REGION 1..12: note = Peptide-112
  SITE 1: note = 3-(2-Naphthyl)-L-alanine
  SITE 11: note = L-Cyclopentylglycine
  SITE 12: note = C-terminal carboxyl group is linked to N-terminal amino group of linker via amide bond
  SITE 1..12: note = Thiol group of cysteine is linked to N-terminal end of 3-(2-Naphthyl)-L-alanine via -CH2-CO-
XRSGRNWVRWXC

SEQ ID NO: 113 - protein, 12 aa, synthetic construct
  REGION 1..12: note = Peptide-113
  SITE 1: note = 3-(2-Naphthyl)-L-alanine
  SITE 5: note = (2S)-2-Amino-4-guanidino-butanoic acid
  SITE 8: note = Nle
  SITE 11: note = L-Cyclopentylglycine
  SITE 12: note = C-terminal carboxyl group is linked to N-terminal amino group of linker via amide bond
  SITE 1..12: note = Thiol group of cysteine is linked to N-terminal end of 3-(2-Naphthyl)-L-alanine via -CH2-CO-
XRSGXNWXRWXC

SEQ ID NO: 114 - protein, 12 aa, synthetic construct
  REGION 1..12: note = Peptide-114
  SITE 1: note = 3-(2-Naphthyl)-L-alanine
  SITE 8: note = Nle
  SITE 11: note = L-Cyclopentylglycine
  SITE 12: note = C-terminal carboxyl group is linked to N-terminal amino group of linker via amide bond
  SITE 1..12: note = Thiol group of cysteine is linked to N-terminal end of 3-(2-Naphthyl)-L-alanine via -CH2-CO-
XRSGRNWXVWXC

SEQ ID NO: 115 - protein, 12 aa, synthetic construct
  REGION 1..12: note = Peptide-115
  SITE 1: note = 3-(2-Naphthyl)-L-alanine
  SITE 5: note = (2S)-2-Amino-4-guanidino-butanoic acid
  SITE 11: note = L-Cyclopentylglycine
  SITE 12: note = C-terminal carboxyl group is linked to N-terminal amino group of linker via amide bond
  SITE 1..12: note = Thiol group of cysteine is linked to N-terminal end of 3-(2-Naphthyl)-L-alanine via -CH2-CO-
XRSGXNWVRWXC

SEQ ID NO: 116 - protein, 12 aa, synthetic construct
  REGION 1..12: note = Peptide-116
  SITE 1: note = 3-(2-Naphthyl)-L-alanine
  SITE 8: note = Nle
  SITE 11: note = L-Alpha-cyclohexylglycine
  SITE 12: note = C-terminal carboxyl group is linked to N-terminal amino group of linker via amide bond
  SITE 1..12: note = Thiol group of cysteine is linked to N-terminal end of 3-(2-Naphthyl)-L-alanine via -CH2-CO-
XRSGRNWXVWXC

SEQ ID NO: 117 - protein, 12 aa, synthetic construct
  REGION 1..12: note = Peptide-117
  SITE 1: note = 3-(2-Naphthyl)-L-alanine
  SITE 2: note = L-Tert-Leucine
  SITE 11: note = L-Cyclopentylglycine
  SITE 12: note = C-terminal carboxyl group is linked to N-terminal amino group of linker via amide bond
  SITE 1..12: note = Thiol group of cysteine is linked to N-terminal end of 3-(2-Naphthyl)-L-alanine via -CH2-CO-
XXSGRNWVRWXC

SEQ ID NO: 118 - protein, 12 aa, synthetic construct
  REGION 1..12: note = Peptide-118
  SITE 1: note = 3-(2-Naphthyl)-L-alanine
  SITE 9: note = (2S)-2-Amino-4-guanidino-butanoic acid
  SITE 11: note = L-Cyclopentylglycine
  SITE 12: note = C-terminal carboxyl group is linked to N-terminal amino group of linker via amide bond
  SITE 1..12: note = Thiol group of cysteine is linked to N-terminal end of 3-(2-Naphthyl)-L-alanine via -CH2-CO-
XRSGRDWVXWXC

SEQ ID NO: 119 - protein, 12 aa, synthetic construct
  REGION 1..12: note = Peptide-119
  SITE 1: note = 3-(2-Naphthyl)-L-alanine
  SITE 5: note = (2S)-2-Amino-4-guanidino-butanoic acid
  SITE 11: note = L-Cyclopentylglycine
  SITE 12: note = C-terminal carboxyl group is linked to N-terminal amino group of linker via amide bond
  SITE 1..12: note = Thiol group of cysteine is linked to N-terminal end of 3-(2-Naphthyl)-L-alanine via -CH2-CO-
XRSGXDWVRWXC

SEQ ID NO: 120 - protein, 12 aa, synthetic construct
  REGION 1..12: note = Peptide-120
  SITE 1: note = 3-(2-Naphthyl)-L-alanine
  SITE 5: note = (2S)-2-Amino-4-guanidino-butanoic acid
  SITE 8: note = Nle
  SITE 11: note = L-Alpha-cyclohexylglycine
  SITE 12: note = C-terminal carboxyl group is linked to N-terminal amino group of linker via amide bond
  SITE 1..12: note = Thiol group of cysteine is linked to N-terminal end of 3-(2-Naphthyl)-L-alanine via -CH2-CO-
XRSGXNWXVWXC

SEQ ID NO: 121 - protein, 12 aa, synthetic construct
  REGION 1..12: note = Peptide-121
  SITE 1: note = 3-(2-Naphthyl)-L-alanine
  SITE 5: note = (2S)-2-Amino-4-guanidino-butanoic acid
  SITE 8: note = Nle
  SITE 11: note = L-Alpha-cyclohexylglycine
  SITE 12: note = C-terminal carboxyl group is linked to N-terminal amino group of linker via amide bond
  SITE 1..12: note = Thiol group of cysteine is linked to N-terminal end of 3-(2-Naphthyl)-L-alanine via -CH2-CO-
XRSGXNWXRWXC

SEQ ID NO: 122 - protein, 12 aa, synthetic construct
  REGION 1..12: note = Peptide-122
  SITE 1: note = 3-(2-Naphthyl)-L-alanine
  SITE 5: note = (2S)-2-Amino-4-guanidino-butanoic acid
  SITE 11: note = L-Alpha-cyclohexylglycine
  SITE 12: note = C-terminal carboxyl group is linked to N-terminal amino group of linker via amide bond
  SITE 1..12: note = Thiol group of cysteine is linked to N-terminal end of 3-(2-Naphthyl)-L-alanine via -CH2-CO-
XRSGXNWVRWXC

SEQ ID NO: 123 - protein, 12 aa, synthetic construct
  REGION 1..12: note = Peptide-123
  SITE 1: note = 3-(2-Naphthyl)-L-alanine
  SITE 5: note = (2S)-2-Amino-4-guanidino-butanoic acid
  SITE 8: note = Nle
  SITE 11: note = L-Cyclopentylglycine
  SITE 12: note = C-terminal carboxyl group is linked to N-terminal amino group of linker via amide bond
  SITE 1..12: note = Thiol group of cysteine is linked to N-terminal end of 3-(2-Naphthyl)-L-alanine via -CH2-CO-
XRSGXDWXRWXC

SEQ ID NO: 124 - DNA, 1422 bp, synthetic construct
  misc_feature 1..1422: note = Nucleotide sequence encoding the heavy chain of anti-LPS mAb-A
  source 1..1422: mol_type = other DNA
  CDS 1..1422: note = Encoding polypeptides including a signal sequence (19 aa)followed by Heavy chain of mAb-A (20-474: 455 aa)
atgaaacacctgtggttcttcctcctgctggtggcagctcccagatgggtgctgagccaggtgcagctggtgcagtctggcgccgaagtgaagaaaccaggcgccagcgtgaaggtgtcctgcaaggccagcggctacacctttaccagctactggatcaactgggtgcgccaggcccctggacagggcctggaatggatgggcaacatctaccccggcagcagcagcatcaactacaacgagaagttcaagagccgcgtgaccatcaccgccgacaccagcacaagcaccgcctacatggaactgagcagcctgcggagcgaggacaccgccgtgtactactgcgcccggaccatctacaactacggcagctccggctacaattacgccatggactactggggccagggcaccctcgtgaccgtgagctcagcctccaccaagggcccaagcgtcttccccctggcaccctcctccaagagcacctctggcggcacagccgccctgggctgcctggtcaaggactacttccccgaacccgtgaccgtgagctggaactcaggcgccctgaccagcggcgtgcacaccttccccgctgtcctgcagtcctcaggactctactccctcagcagcgtggtgaccgtgccctccagcagcttgggcacccagacctacatctgcaacgtgaatcacaagcccagcaacaccaaggtggacaagagagttgagcccaaatcttgtgacaaaactcacacatgcccaccctgcccagcacctgaactcctggggggaccctcagtcttcctcttccccccaaaacccaaggacaccctcatgatctcccggacccctgaggtcacatgcgtggtggtggacgtgagccacgaagaccctgaggtcaagttcaactggtacgtggacggcgtggaggtgcataatgccaagacaaagccccgggaggagcagtacaacagcacgtaccgggtggtcagcgtcctcaccgtcctgcaccaggactggctgaatggcaaggagtacaagtgcaaggtctccaacaaagccctcccagcccccatcgagaaaaccatctccaaagccaaaggccagccccgggaaccacaggtgtacaccctgcccccatcccgggaggagatgaccaagaaccaggtcagcctgacctgcctggtcaaaggcttctatcccagcgacatcgccgtggagtgggagagcaatggccagcccgagaacaactacaagaccacccctcccgtgctggactccgacggctccttcttcctctacagcaagctcaccgtggacaagagcaggtggcagcagggcaacgtcttctcatgctccgtgatgcatgaggctctgcacaaccactacacccagaagagcctctccctgtctcccggcaaa

SEQ ID NO: 125 - protein, 474 aa, synthetic construct
  REGION 1..474: note = Synthetic Construct
MKHLWFFLLLVAAPRWVLSQVQLVQSGAEVKKPGASVKVSCKASGYTFTSYWINWVRQAPGQGLEWMGNIYPGSSSINYNEKFKSRVTITADTSTSTAYMELSSLRSEDTAVYYCARTIYNYGSSGYNYAMDYWGQGTLVTVSSASTKGPSVFPLAPSSKSTSGGTAALGCLVKDYFPEPVTVSWNSGALTSGVHTFPAVLQSSGLYSLSSVVTVPSSSLGTQTYICNVNHKPSNTKVDKRVEPKSCDKTHTCPPCPAPELLGGPSVFLFPPKPKDTLMISRTPEVTCVVVDVSHEDPEVKFNWYVDGVEVHNAKTKPREEQYNSTYRVVSVLTVLHQDWLNGKEYKCKVSNKALPAPIEKTISKAKGQPREPQVYTLPPSREEMTKNQVSLTCLVKGFYPSDIAVEWESNGQPENNYKTTPPVLDSDGSFFLYSKLTVDKSRWQQGNVFSCSVMHEALHNHYTQKSLSLSPGK

SEQ ID NO: 126 - DNA, 702 bp, synthetic construct
  misc_feature 1..702: note = Nucleotide sequence encoding the light chain of anti-LPS mAb-A
  source 1..702: mol_type = other DNA
  CDS 1..702: note = Encoding polypeptides including a signal sequence (20 aa)followed by light chain of mAb-A (21-234: 214 aa)
atggtgctgcagacccaggtgttcatctccctgctgctgtggatctccggcgcgtacggcgacatcgtgatgacccagagccctgacagcctggccgtgtctctgggagagagagccaccatcaactgcaaggccagcgagaacgtgggcaacagcgtgtcctggtatcagcagaagcccggccagccccccaagctgctgatctacggcgccagcaacagatacaccggcgtgcccgatagattcagcggcagcggctctggcaccgacttcaccctgacaatcagctccctgcaggccgaggacgtggccgtgtactactgtggccagagctacagctacccctacaccttcggccagggcaccaaggtggaaatcaagcgtacggtggccgccccctccgtgttcatcttccccccctccgacgagcagctgaagtccggcaccgcctccgtggtgtgcctgctgaataacttctaccccagagaggccaaggtgcagtggaaggtggacaacgccctgcagtccgggaactcccaggagagcgtgaccgagcaggacagcaaggacagcacctacagcctgagcagcaccctgaccctgagcaaagccgactacgagaagcacaaggtgtacgcctgcgaggtgacccaccagggcctgagctcccccgtcaccaagagcttcaacaggggggagtgt

SEQ ID NO: 127 - protein, 234 aa, synthetic construct
  REGION 1..234: note = Synthetic Construct
MVLQTQVFISLLLWISGAYGDIVMTQSPDSLAVSLGERATINCKASENVGNSVSWYQQKPGQPPKLLIYGASNRYTGVPDRFSGSGSGTDFTLTISSLQAEDVAVYYCGQSYSYPYTFGQGTKVEIKRTVAAPSVFIFPPSDEQLKSGTASVVCLLNNFYPREAKVQWKVDNALQSGNSQESVTEQDSKDSTYSLSSTLTLSKADYEKHKVYACEVTHQGLSSPVTKSFNRGEC

SEQ ID NO: 128 - DNA, 1097 bp, synthetic construct
  misc_feature 1..1097: note = Nucleotide sequence encoding the heavy chain of CLCH-A
  source 1..1097: mol_type = other DNA
  CDS 26..1072: note = Encoding polypeptides including a signal sequence (19 aa)followed by CH-A (20-349: 330 aa)
ccagcctccggactctagagccaccatgaagcacctgtggttctttctgctgctggtggccgctcccagatgggtgctgagcgcctctacaaagggccccagcgtgttccctctggcccctagcagcaagagcacatctggcggaacagccgccctgggctgcctcgtgaaggactactttcccgagcccgtgaccgtgtcctggaactctggcgctctgacaagcggcgtgcacacctttccagccgtgctgcagagcagcggcctgtactctctgagcagcgtcgtgacagtgcccagcagctctctgggcacccagacctacatctgcaacgtgaaccacaagcccagcaacaccaaggtggacaagcgggtggaacccaagagctgcgacaagacccacacctgtcccccttgtcctgcccccgaactgctgggaggcccttccgtgttcctgttccccccaaagcccaaggacaccctgatgatcagccggacccccgaagtgacctgcgtggtggtggatgtgtcccacgaggaccctgaagtgaagttcaattggtacgtggacggcgtggaagtgcacaacgccaagaccaagcctagagaggaacagtacaacagcacctaccgggtggtgtccgtgctgacagtgctgcaccaggactggctgaacggcaaagagtacaagtgcaaggtgtccaacaaggccctgcctgcccccatcgagaaaaccatcagcaaggccaagggccagccccgcgaaccccaggtgtacacactgcccccaagccgggaagagatgaccaagaaccaggtgtccctgacctgtctcgtgaaaggcttctacccctccgatatcgccgtggaatgggagagcaacggccagcccgagaacaactacaagaccaccccccctgtgctggacagcgacggctcattcttcctgtacagcaagctgaccgtggacaagagccggtggcagcagggcaacgtgttcagctgcagcgtgatgcacgaggccctgcacaaccactacacccagaagtccctgagcctgagccccggcaaatgagtttaaacgggggaggctaact

SEQ ID NO: 129 - protein, 349 aa, synthetic construct
  REGION 1..349: note = Synthetic Construct
MKHLWFFLLLVAAPRWVLSASTKGPSVFPLAPSSKSTSGGTAALGCLVKDYFPEPVTVSWNSGALTSGVHTFPAVLQSSGLYSLSSVVTVPSSSLGTQTYICNVNHKPSNTKVDKRVEPKSCDKTHTCPPCPAPELLGGPSVFLFPPKPKDTLMISRTPEVTCVVVDVSHEDPEVKFNWYVDGVEVHNAKTKPREEQYNSTYRVVSVLTVLHQDWLNGKEYKCKVSNKALPAPIEKTISKAKGQPREPQVYTLPPSREEMTKNQVSLTCLVKGFYPSDIAVEWESNGQPENNYKTTPPVLDSDGSFFLYSKLTVDKSRWQQGNVFSCSVMHEALHNHYTQKSLSLSPGK

SEQ ID NO: 130 - DNA, 425 bp, synthetic construct
  misc_feature 1..425: note = Nucleotide sequence encoding the light chain of CLCH-A
  source 1..425: mol_type = other DNA
  CDS 26..400: note = Encoding polypeptides including a signal sequence (20 aa)followed by CL-A (21-125: 105 aa)
ccagcctccggactctagagccaccatggtgctgcagacccaggtgttcatcagcctgctgctgtggatcagcggcgcctatggcgtggcagcccctagcgtgttcatcttcccacccagcgacgagcagctgaagtctggcacagccagcgtcgtgtgcctgctgaacaacttctacccccgcgaggccaaggtgcagtggaaggtggacaatgccctgcagagcggcaacagccaggaaagcgtgaccgagcaggacagcaaggactccacctacagcctgagcagcaccctgaccctgagcaaggccgactacgagaagcacaaggtgtacgcctgcgaagtgacccaccagggcctgtctagccccgtgaccaagagcttcaaccggggcgagtgttgagtttaaacgggggaggctaact

SEQ ID NO: 131 - protein, 125 aa, synthetic construct
  REGION 1..125: note = Synthetic Construct
MVLQTQVFISLLLWISGAYGVAAPSVFIFPPSDEQLKSGTASVVCLLNNFYPREAKVQWKVDNALQSGNSQESVTEQDSKDSTYSLSSTLTLSKADYEKHKVYACEVTHQGLSSPVTKSFNRGEC

SEQ ID NO: 132 - DNA, 1047 bp, synthetic construct
  misc_feature 1..1047: note = Nucleotide sequence encoding the heavy chain of CLCH-B (LALAform)
  source 1..1047: mol_type = other DNA
  CDS 1..1047: note = Encoding polypeptides including a signal sequence (19 aa)followed by CH-B (20-349: 330 aa)
atgaagcacctgtggttctttctgctgctggtggccgctcccagatgggtgctgagcgcctctacaaagggccccagcgtgttccctctggcccctagcagcaagagcacatctggcggaacagccgccctgggctgcctcgtgaaggactactttcccgagcccgtgaccgtgtcctggaactctggcgctctgacaagcggcgtgcacacctttccagccgtgctgcagagcagcggcctgtactctctgagcagcgtcgtgacagtgcccagcagctctctgggcacccagacctacatctgcaacgtgaaccacaagcccagcaacaccaaggtggacaagcgggtggaacccaagagctgcgacaagacccacacctgtcccccttgtcctgcccccgaagccgcgggaggcccttccgtgttcctgttccccccaaagcccaaggacaccctgatgatcagccggacccccgaagtgacctgcgtggtggtggatgtgtcccacgaggaccctgaagtgaagttcaattggtacgtggacggcgtggaagtgcacaacgccaagaccaagcctagagaggaacagtacaacagcacctaccgggtggtgtccgtgctgacagtgctgcaccaggactggctgaacggcaaagagtacaagtgcaaggtgtccaacaaggccctgcctgcccccatcgagaaaaccatcagcaaggccaagggccagccccgcgaaccccaggtgtacacactgcccccaagccgggaagagatgaccaagaaccaggtgtccctgacctgtctcgtgaaaggcttctacccctccgatatcgccgtggaatgggagagcaacggccagcccgagaacaactacaagaccaccccccctgtgctggacagcgacggctcattcttcctgtacagcaagctgaccgtggacaagagccggtggcagcagggcaacgtgttcagctgcagcgtgatgcacgaggccctgcacaaccactacacccagaagtccctgagcctgagccccggcaaa

SEQ ID NO: 133 - protein, 349 aa, synthetic construct
  REGION 1..349: note = Synthetic Construct
MKHLWFFLLLVAAPRWVLSASTKGPSVFPLAPSSKSTSGGTAALGCLVKDYFPEPVTVSWNSGALTSGVHTFPAVLQSSGLYSLSSVVTVPSSSLGTQTYICNVNHKPSNTKVDKRVEPKSCDKTHTCPPCPAPEAAGGPSVFLFPPKPKDTLMISRTPEVTCVVVDVSHEDPEVKFNWYVDGVEVHNAKTKPREEQYNSTYRVVSVLTVLHQDWLNGKEYKCKVSNKALPAPIEKTISKAKGQPREPQVYTLPPSREEMTKNQVSLTCLVKGFYPSDIAVEWESNGQPENNYKTTPPVLDSDGSFFLYSKLTVDKSRWQQGNVFSCSVMHEALHNHYTQKSLSLSPGK

SEQ ID NO: 134 - DNA, 779 bp, synthetic construct
  misc_feature 1..779: note = Nucleotide sequence encoding Fc fragment (wild type)
  source 1..779: mol_type = other DNA
  CDS 26..754: note = Encoding polypeptide containing a signal sequence (20 aa)followed by Fc-B (223 aa)
ccagcctccggactctagagccaccatggtgctgcagacccaggtgttcatcagcctgctgctgtggatcagcggcgcctacggcacctgtcctccatgtcctgctccagagctgctgggcggacctagcgtgttcctgttccccccaaagcccaaggacaccctgatgatcagccggacccccgaagtgacctgcgtggtggtggatgtgtcccacgaggaccctgaagtgaagttcaattggtacgtggacggcgtggaagtgcacaacgccaagaccaagcccagagaggaacagtacaacagcacctaccgggtggtgtccgtgctgaccgtgctgcaccaggactggctgaacggcaaagagtacaagtgcaaggtgtccaacaaggccctgcctgcccccatcgagaaaaccatcagcaaggccaagggccagccccgcgaaccccaggtgtacacactgccccctagcagggacgagctgaccaagaaccaggtgtccctgacctgtctcgtgaagggcttctacccctccgatatcgccgtggaatgggagagcaacggccagcccgagaacaactacaagaccaccccccctgtgctggacagcgacggctcattcttcctgtacagcaagctgacagtggacaagagccggtggcagcagggcaacgtgttcagctgcagcgtgatgcacgaggccctgcacaaccactacacccagaagtccctgagcctgagccccggcaaatgagtttaaacgggggaggctaact

SEQ ID NO: 135 - protein, 243 aa, synthetic construct
  REGION 1..243: note = Synthetic Construct
MVLQTQVFISLLLWISGAYGTCPPCPAPELLGGPSVFLFPPKPKDTLMISRTPEVTCVVVDVSHEDPEVKFNWYVDGVEVHNAKTKPREEQYNSTYRVVSVLTVLHQDWLNGKEYKCKVSNKALPAPIEKTISKAKGQPREPQVYTLPPSRDELTKNQVSLTCLVKGFYPSDIAVEWESNGQPENNYKTTPPVLDSDGSFFLYSKLTVDKSRWQQGNVFSCSVMHEALHNHYTQKSLSLSPGK

SEQ ID NO: 136 - DNA, 741 bp, synthetic construct
  misc_feature 1..741: note = Nucleotide sequence encoding Fc-A (LALA form)
  source 1..741: mol_type = other DNA
  CDS 1..741: note = Encoding a signal peptide (20 aa) and Fc-A (227 aa)
atggtgctgcagacccaggtgttcatcagcctgctgctgtggatcagcggcgcctacggcgacaaaactcacacctgtcctccatgtcctgctccagaggccgcgggcggacctagcgtgttcctgttccccccaaagcccaaggacaccctgatgatcagccggacccccgaagtgacctgcgtggtggtggatgtgtcccacgaggaccctgaagtgaagttcaattggtacgtggacggcgtggaagtgcacaacgccaagaccaagcccagagaggaacagtacaacagcacctaccgggtggtgtccgtgctgaccgtgctgcaccaggactggctgaacggcaaagagtacaagtgcaaggtgtccaacaaggccctgcctgcccccatcgagaaaaccatcagcaaggccaagggccagccccgcgaaccccaggtgtacacactgccccctagcagggacgagctgaccaagaaccaggtgtccctgacctgtctcgtgaagggcttctacccctccgatatcgccgtggaatgggagagcaacggccagcccgagaacaactacaagaccaccccccctgtgctggacagcgacggctcattcttcctgtacagcaagctgacagtggacaagagccggtggcagcagggcaacgtgttcagctgcagcgtgatgcacgaggccctgcacaaccactacacccagaagtccctgagcctgagccccggcaaa

SEQ ID NO: 137 - protein, 247 aa, synthetic construct
  REGION 1..247: note = Synthetic Construct
MVLQTQVFISLLLWISGAYGDKTHTCPPCPAPEAAGGPSVFLFPPKPKDTLMISRTPEVTCVVVDVSHEDPEVKFNWYVDGVEVHNAKTKPREEQYNSTYRVVSVLTVLHQDWLNGKEYKCKVSNKALPAPIEKTISKAKGQPREPQVYTLPPSRDELTKNQVSLTCLVKGFYPSDIAVEWESNGQPENNYKTTPPVLDSDGSFFLYSKLTVDKSRWQQGNVFSCSVMHEALHNHYTQKSLSLSPGK

SEQ ID NO: 138 - DNA, 791 bp, synthetic construct
  misc_feature 1..791: note = DNA fragment containing nucleotide sequence encoding Fc-C (LALA-PA form)
  source 1..791: mol_type = other DNA
  CDS 26..766: note = Encoding a signal peptide (20 aa) and Fc-C (227 aa)
ccagcctccggactctagagccaccatggtgctgcagacccaggtgttcatcagcctgctgctgtggatctctggcgcctacggcgataagacccacacctgtcctccatgtcctgctccagaagctgctggcggcccttccgtgtttctgttccctccaaagcctaaggacaccctgatgatcagcagaacccctgaagtgacctgcgtggtggtggatgtgtcccacgaggatcccgaagtgaagttcaattggtacgtggacggcgtggaagtgcacaacgccaagaccaagcctagagaggaacagtacaacagcacctacagagtggtgtccgtgctgaccgtgctgcaccaggattggctgaacggcaaagagtacaagtgcaaggtgtccaacaaggccctggccgctcctatcgagaaaaccatcagcaaggccaagggccagcctagggaaccccaggtttacacactgcctccaagccgggaagagatgaccaagaaccaggtgtccctgacctgcctggtcaagggcttctacccttccgatatcgccgtggaatgggagagcaatggccagcctgagaacaactacaagaccacacctcctgtgctggacagcgacggctcattcttcctgtacagcaagctgacagtggacaagagcagatggcagcagggcaacgtgttcagctgcagcgtgatgcacgaggccctgcacaaccactacacccagaagtccctgagcctgtctcctggcaaatgagtttaaacgggggaggctaact

SEQ ID NO: 139 - protein, 247 aa, synthetic construct
  REGION 1..247: note = Synthetic Construct
MVLQTQVFISLLLWISGAYGDKTHTCPPCPAPEAAGGPSVFLFPPKPKDTLMISRTPEVTCVVVDVSHEDPEVKFNWYVDGVEVHNAKTKPREEQYNSTYRVVSVLTVLHQDWLNGKEYKCKVSNKALAAPIEKTISKAKGQPREPQVYTLPPSREEMTKNQVSLTCLVKGFYPSDIAVEWESNGQPENNYKTTPPVLDSDGSFFLYSKLTVDKSRWQQGNVFSCSVMHEALHNHYTQKSLSLSPGK

SEQ ID NO: 140 - protein, 4 aa, synthetic construct
  REGION 1..4: note = Linker L1
GGGG

SEQ ID NO: 141 - protein, 4 aa, synthetic construct
  REGION 1..4: note = Linker L1
GSGS

SEQ ID NO: 142-143 - skipped (2 entries)

SEQ ID NO: 144 - protein, 5 aa, synthetic construct
  REGION 1..5: note = Linker L1
GGEGG

SEQ ID NO: 145-147 - skipped (3 entries)

SEQ ID NO: 148 - protein, 232 aa, synthetic construct
  REGION 1..232: note = Polypeptide consisting of hinge, CH2 domain, and CH3 domain ofhuman IgG heavy chain
EPKSCDKTHTCPPCPAPELLGGPSVFLFPPKPKDTLMISRTPEVTCVVVDVSHEDPEVKFNWYVDGVEVHNAKTKPREEQYNSTYRVVSVLTVLHQDWLNGKEYKCKVSNKALPAPIEKTISKAKGQPREPQVYTLPPSRDELTKNQVSLTCLVKGFYPSDIAVEWESNGQPENNYKTTPPVLDSDGSFFLYSKLTVDKSRWQQGNVFSCSVMHEALHNHYTQKSLSLSPGK

SEQ ID NO: 149 - protein, 12 aa, synthetic construct
  REGION 1..12: note = Peptide-124
  SITE 1: note = 3-(2-Naphthyl)-L-alanine
  SITE 11: note = L-Cyclopentylglycine
  SITE 1..12: note = Thiol group of cysteine is linked to N-terminal end of 3-(2-Naphthyl)-L-alanine via -CH2-CO-
  SITE 12: note = C-terminal carboxyl group is linked to N-terminal amino group of linker via amide bond
XRSGRDWVRWXC

SEQ ID NO: 150 - protein, 12 aa, synthetic construct
  REGION 1..12: note = Peptide-125
  SITE 1: note = 3-(2-Naphthyl)-L-alanine
  SITE 3: note = L-Homocysteine
  SITE 8: note = L-Homocysteine
  SITE 11: note = L-Cyclopentylglycine
  SITE 12: note = Amidation of C-terminal carboxyl group
  SITE 1..12: note = Thiol group of cysteine is linked to N-terminal end of 3-(2-Naphthyl)-L-alanine via -CH2-CO-
  SITE 3..8: note = Thiol groups are linked as -S-CH2-CO-CH2-S-
XRXGRDWXRWXC

SEQ ID NO: 151 - protein, 12 aa, synthetic construct
  REGION 1..12: note = Peptide-126
  SITE 1: note = 3-(2-Naphthyl)-L-alanine
  SITE 8: note = L-Homocysteine
  SITE 11: note = L-Cyclopentylglycine
  SITE 12: note = Amidation of C-terminal carboxyl group
  SITE 1..12: note = Thiol group of cysteine is linked to N-terminal end of 3-(2-Naphthyl)-L-alanine via -CH2-CO-
  SITE 3..8: note = Thiol groups are linked as a disulfide
XRCGRDWXRWXC

SEQ ID NO: 152 - protein, 12 aa, synthetic construct
  REGION 1..12: note = Peptide-127
  SITE 1: note = 3-(2-Naphthyl)-L-alanine
  SITE 3: note = L-Homocysteine
  SITE 8: note = L-Homocysteine
  SITE 11: note = L-Cyclopentylglycine
  SITE 12: note = Amidation of C-terminal carboxyl group
  SITE 1..12: note = Thiol group of cysteine is linked to N-terminal end of 3-(2-Naphthyl)-L-alanine via -CH2-CO-
  SITE 3..8: note = Thiol groups are linked as -S-CH2-S-
XRXGRDWXRWXC

SEQ ID NO: 153 - protein, 12 aa, synthetic construct
  REGION 1..12: note = Peptide-128
  SITE 1: note = 3-(2-Naphthyl)-L-alanine
  SITE 11: note = L-Cyclopentylglycine
  SITE 12: note = Amidation of C-terminal carboxyl group
  SITE 1..12: note = Thiol group of cysteine is linked to N-terminal end of 3-(2-Naphthyl)-L-alanine via -CH2-CO-
  SITE 3..8: note = Thiol groups are linked as a disulfide
XRCGRDWCRWXC

SEQ ID NO: 154 - protein, 12 aa, synthetic construct
  REGION 1..12: note = Peptide-129
  SITE 1: note = 3-(2-Naphthyl)-L-alanine
  SITE 3: note = L-Homocysteine
  SITE 11: note = L-Cyclopentylglycine
  SITE 12: note = Amidation of C-terminal carboxyl group
  SITE 1..12: note = Thiol group of cysteine is linked to N-terminal end of 3-(2-Naphthyl)-L-alanine via -CH2-CO-
  SITE 3..8: note = Thiol groups are linked as a disulfide
XRXGRDWCRWXC

SEQ ID NO: 155 - protein, 12 aa, synthetic construct
  REGION 1..12: note = Peptide-130
  SITE 1: note = 3-(2-Naphthyl)-L-alanine
  SITE 11: note = L-Cyclopentylglycine
  SITE 12: note = Amidation of C-terminal carboxyl group
  SITE 1..12: note = Thiol group of cysteine is linked to N-terminal end of 3-(2-Naphthyl)-L-alanine via -CH2-CO-
  SITE 3..8: note = Thiol groups are linked as -S-CH2-S-
XRCGRDWCRWXC

SEQ ID NO: 156 - protein, 12 aa, synthetic construct
  REGION 1..12: note = Peptide-131
  SITE 1: note = 3-(2-Naphthyl)-L-alanine
  SITE 8: note = L-Homocysteine
  SITE 11: note = L-Cyclopentylglycine
  SITE 12: note = Amidation of C-terminal carboxyl group
  SITE 1..12: note = Thiol group of cysteine is linked to N-terminal end of 3-(2-Naphthyl)-L-alanine via -CH2-CO-
  SITE 3..8: note = Thiol groups are linked as -S-CH2-S-
XRCGRDWXRWXC

SEQ ID NO: 157 - protein, 12 aa, synthetic construct
  REGION 1..12: note = Peptide-132
  SITE 1: note = 3-(2-Naphthyl)-L-alanine
  SITE 3: note = L-Homocysteine
  SITE 11: note = L-Cyclopentylglycine
  SITE 12: note = Amidation of C-terminal carboxyl group
  SITE 1..12: note = Thiol group of cysteine is linked to N-terminal end of 3-(2-Naphthyl)-L-alanine via -CH2-CO-
  SITE 3..8: note = Thiol groups are linked as -S-CH2-S-
XRXGRDWCRWXC

SEQ ID NO: 158 - protein, 12 aa, synthetic construct
  REGION 1..12: note = Peptide-133
  SITE 1: note = 3-(2-Naphthyl)-L-alanine
  SITE 8: note = L-Homocysteine
  SITE 11: note = L-Cyclopentylglycine
  SITE 12: note = Amidation of C-terminal carboxyl group
  SITE 1..12: note = Thiol group of cysteine is linked to N-terminal end of 3-(2-Naphthyl)-L-alanine via -CH2-CO-
  SITE 3: note = L-Penicillamine
  SITE 3..8: note = Thiol groups are linked as -S-CH2-S-
XRXGRDWXRWXC

SEQ ID NO: 159 - protein, 12 aa, synthetic construct
  REGION 1..12: note = Peptide-134
  SITE 1: note = 3-(2-Naphthyl)-L-alanine
  SITE 3: note = L-Homocysteine
  SITE 11: note = L-Cyclopentylglycine
  SITE 12: note = Amidation of C-terminal carboxyl group
  SITE 1..12: note = Thiol group of cysteine is linked to N-terminal end of 3-(2-Naphthyl)-L-alanine via -CH2-CO-
  SITE 3..8: note = Thiol groups are linked as a disulfide
  SITE 8: note = L-Penicillamine
XRXGRDWXRWXC

SEQ ID NO: 160 - protein, 12 aa, synthetic construct
  REGION 1..12: note = Peptide-135
  SITE 1: note = 3-(2-Naphthyl)-L-alanine
  SITE 8: note = L-Homocysteine
  SITE 11: note = L-Cyclopentylglycine
  SITE 12: note = Amidation of C-terminal carboxyl group
  SITE 1..12: note = Thiol group of cysteine is linked to N-terminal end of 3-(2-Naphthyl)-L-alanine via -CH2-CO-
  SITE 3..8: note = Thiol groups are linked as a disulfide
  SITE 3: note = L-Penicillamine
XRXGRDWXRWXC

SEQ ID NO: 161 - protein, 12 aa, synthetic construct
  REGION 1..12: note = Peptide-136
  SITE 1: note = 3-(2-Naphthyl)-L-alanine
  SITE 3: note = L-Homocysteine
  SITE 11: note = L-Cyclopentylglycine
  SITE 12: note = Amidation of C-terminal carboxyl group
  SITE 1..12: note = Thiol group of cysteine is linked to N-terminal end of 3-(2-Naphthyl)-L-alanine via -CH2-CO-
  SITE 8: note = L-Penicillamine
  SITE 3..8: note = Thiol groups are linked as -S-CH2-S-
XRXGRDWXRWXC

SEQ ID NO: 162 - protein, 12 aa, synthetic construct
  REPEAT 1..12: note = Peptide-137
  SITE 1: note = 3-(2-Naphthyl)-L-alanine
  SITE 11: note = L-Cyclopentylglycine
  SITE 12: note = Amidation of C-terminal carboxyl group
  SITE 1..12: note = Thiol group of cysteine is linked to N-terminal end of 3-(2-Naphthyl)-L-alanine via -CH2-CO-
  SITE 3: note = L-Penicillamine
  SITE 3..8: note = Thiol groups are linked as -S-CH2-S-
XRXGRDWCRWXC

SEQ ID NO: 163 - protein, 12 aa, synthetic construct
  REGION 1..12: note = Peptide-138
  SITE 1: note = 3-(2-Naphthyl)-L-alanine
  SITE 11: note = L-Cyclopentylglycine
  SITE 12: note = Amidation of C-terminal carboxyl group
  SITE 1..12: note = Thiol group of cysteine is linked to N-terminal end of 3-(2-Naphthyl)-L-alanine via -CH2-CO-
  SITE 3..8: note = Thiol groups are linked as a disulfide
  SITE 8: note = L-Penicillamine
XRCGRDWXRWXC

SEQ ID NO: 164 - protein, 12 aa, synthetic construct
  REGION 1..12: note = Peptide-139
  SITE 1: note = 3-(2-Naphthyl)-L-alanine
  SITE 11: note = L-Cyclopentylglycine
  SITE 12: note = Amidation of C-terminal carboxyl group
  SITE 1..12: note = Thiol group of cysteine is linked to N-terminal end of 3-(2-Naphthyl)-L-alanine via -CH2-CO-
  SITE 8: note = L-Penicillamine
  SITE 3..8: note = Thiol groups are linked as -S-CH2-S-
XRCGRDWXRWXC

SEQ ID NO: 165 - DNA, 741 bp, synthetic construct
  source 1..741: mol_type = other DNA
  misc_feature 1..741: note = Nucleotide sequence encoding Fc-C (LALA-PA form)
  CDS 1..741: note = Nucleotide sequence encoding Fc-C (LALA-PA form); protein_id = 166; translation = MVLQTQVFISLLLWISGAYGDKTHTCPPCPAPEAAGGPSVFLFPPKPKDTLMISRTPEVTCVVVDVSHEDPEVKFNWYVDGVEVHNAKTKPREEQYNSTYRVVSVLTVLHQDWLNGKEYKCKVSNKALAAPIEKTISKAKGQPREPQVYTLPPSREEMTKNQVSLTCLVKGFYPSDIAVEWESNGQPENNYKTTPPVLDSDGSFFLYSKLTVDKSRWQQGNVFSCSVMHEALHNHYTQKSLSLSPGK
atggtgctgcagacccaggtgttcatcagcctgctgctgtggatctctggcgcctacggcgataagacccacacctgtcctccatgtcctgctccagaagctgctggcggcccttccgtgtttctgttccctccaaagcctaaggacaccctgatgatcagcagaacccctgaagtgacctgcgtggtggtggatgtgtcccacgaggatcccgaagtgaagttcaattggtacgtggacggcgtggaagtgcacaacgccaagaccaagcctagagaggaacagtacaacagcacctacagagtggtgtccgtgctgaccgtgctgcaccaggattggctgaacggcaaagagtacaagtgcaaggtgtccaacaaggccctggccgctcctatcgagaaaaccatcagcaaggccaagggccagcctagggaaccccaggtttacacactgcctccaagccgggaagagatgaccaagaaccaggtgtccctgacctgcctggtcaagggcttctacccttccgatatcgccgtggaatgggagagcaatggccagcctgagaacaactacaagaccacacctcctgtgctggacagcgacggctcattcttcctgtacagcaagctgacagtggacaagagcagatggcagcagggcaacgtgttcagctgcagcgtgatgcacgaggccctgcacaaccactacacccagaagtccctgagcctgtctcctggcaaa

SEQ ID NO: 166 - protein, 247 aa, synthetic construct; identical to SEQ ID NO: 139